European Patent Specification EP 3 354 730 B1, published June 18, 2025. Title: Method of Producing Linalool. Applicant: Ajinomoto Co., Inc. The sequence listing filed with the application follows.

SEQUENCE LISTING (183 sequences)

SEQ ID NO: 1 - protein, 574 aa, Actinidia arguta
MASFNRFCVSSLLAPNNSPQISNAPRSTAVPSMPTTQKWSITEDLAFISNPSKQHNHQTGYRIFSDEFYLKHENKLKDVRRALREVEETPLEGLVMIDTLQRLGIDYHFQGEIGALLQKQQRISTCDYPEHDLFEVSTRFRLLRQEGHNVPADVFNNFRDKEGRFKSELSRDIRGLMSLYEASQLSIQGEDILDQAADFSSQLLSGWATNLDHHQARLVRNALTHPYHKSLATFMARNFNYDCKGQNGWVNNLQELAKMDLTMVQSMHQKEVLQVSQWWKGRGLANELKLVRNQPLKWYMWPMAALTDPRFSEERVELTKPISFIYIIDDIFDVYGTLEELTLFTDAVNRWELTAVEQLPDYMKICFKALYDITNEIAYKIYKKHGRNPIDSLRRTWASLCNAFLEEAKWFASGNLPKAEEYLKNGIISSGMHVVTVHMFFLLGGCFTEESVNLVDEHAGITSSIATILRLSDDLGSAKDEDQDGYDGSYLECYLKDHKGSSVENAREEVIRMISDAWKRLNEECLFPNPFSATFRKGSLNIARMVPLMYSYDDNHNLPILEEHMKTMLYDSSS

SEQ ID NO: 2 - DNA, 1725 bp, Actinidia arguta
atggccagcttcaacaggttttgtgtctcttctcttcttgctccaaacaacagcccacaaattagcaatgctccccgctccaccgctgtaccctctatgcctaccacccaaaaatggagcatcaccgaagacctagcattcatttctaatccctcgaaacaacacaaccatcaaaccggatatcgcattttctctgatgagttttacctaaagcacgaaaacaaattgaaggacgttaggagagcgttaagggaagtggaggaaaccccattagaaggtctggtcatgatcgacaccctccaacggctaggcattgactaccacttccagggggagattggagccctactacagaaacaacagagaatatctacttgtgattatcccgagcatgatctttttgaggtctctactcgctttcggctgttaaggcaagaaggtcacaatgtgcctgcagatgtgtttaacaacttcagagacaaggagggaaggttcaaatcagaactaagcagagacatcagggggttgatgagtttgtatgaagcttcacagttaagcatacaaggagaagacatacttgatcaagccgcagattttagttcccaactccttagcgggtgggcgacaaatctcgatcatcatcaagctaggcttgtgcgtaatgcactgacacatccctatcacaagagcctagcgacattcatggcaagaaacttcaattatgattgcaagggccaaaatggatgggtcaataacttgcaagaactagcaaaaatggacttaactatggttcagtccatgcatcaaaaagaagtccttcaagtttcccaatggtggaaaggcaggggtttggccaatgaattgaagcttgtgagaaatcagccacttaaatggtacatgtggccaatggcagccctcacagatccaagattctcagaggaaagagttgaactcacaaaaccaatctcttttatctatatcatagatgacatttttgatgtttatgggacattagaagaactcactctcttcacagatgctgtcaatagatgggaacttactgctgttgagcaactacccgactacatgaagatttgctttaaggctctttatgacatcacaaatgaaatcgcctacaagatctacaaaaagcatggacggaaccccatagattctctgcggagaacgtgggcaagtttgtgcaacgcgttcttagaagaagcaaaatggtttgcttctgggaacttgccaaaggcagaagagtacttgaagaatgggatcatcagttcagggatgcatgtggttacggttcacatgttctttctcttgggcggttgtttcaccgaagaaagtgtcaatcttgtggatgaacatgcgggaattacatcttctatagcaacaatccttcgtctttcggatgacttgggaagtgccaaggatgaggatcaagatggctacgatggatcctatttagaatgctatctgaaggaccacaagggctcttcggtagagaatgcaagagaagaagttattcgcatgatttcagatgcatggaagcgcctcaacgaggaatgcctatttccgaatccattttcagcaactttcaggaagggttctcttaatatcgcaaggatggttcctttgatgtacagctatgatgacaatcataacctcccaatccttgaggagcacatgaagacaatgctctatgatagttcttcttga

SEQ ID NO: 3 - DNA, 1650 bp, Artificial Sequence
  DNA having modified codons, which encodes linalool synthase gene derived from Actinidia arguta (opt_AaLINS)
atgtccaccgccgtgccctctatgcccactacccaaaaatggtctattaccgaagacttagcctttattagcaatcccagcaaacaacataatcaccaaaccggctaccggatttttagtgacgaattttacctgaaacatgaaaacaaattgaaagatgtgcggcgcgccttgcgtgaagttgaagaaacccccctggaaggcttggtgatgattgacactttacagcggctgggtattgattaccactttcaaggcgaaattggtgccttgttacagaaacaacagcgcattagtacctgtgactatcccgaacatgatttgtttgaagtgagcactcgctttcgtctgttgcgtcaagaaggtcacaatgtgcccgccgacgtttttaataactttcgcgataaagaagggcgttttaaatctgaactgtcccgggatattcgcggattgatgtccttatacgaagccagtcaactgagcattcagggggaagacattttggatcaagccgctgacttttccagtcagttactgtctggatgggccaccaatttagatcatcaccaagcccgtctggtgcggaacgctttgacccatccctaccacaaaagtctggccacttttatggctcgcaactttaactacgattgcaaagggcaaaacggatgggtgaataacctgcaggaattggccaaaatggatttaaccatggttcaaagtatgcatcagaaagaagtgctgcaagttagccagtggtggaaagggcggggattggccaatgaactgaaattggtgcgcaaccaacccttgaaatggtatatgtggcccatggccgctttaaccgatccccggttttctgaagaacgcgtggaattgactaaacccatttcctttatttacattattgatgacatttttgacgtttatggcaccttagaagaattaaccctgtttactgatgccgtgaatcggtgggaattaactgctgttgaacagctgcccgactacatgaaaatttgttttaaagccttgtacgatattaccaacgaaattgcttacaaaatttacaaaaaacatgggcgcaaccccattgatagtttacgtcggacttgggccagcttatgcaatgcttttctggaagaagccaaatggtttgctagtggcaatttgcccaaagccgaagaatacctgaaaaacgggattattagctctggaatgcatgtggttaccgtgcacatgtttttcttgttaggcggttgttttactgaagaatccgtgaatttggttgatgaacatgccggcattacctccagtattgctactattttgcgtttatctgatgacttaggttccgccaaagatgaagaccaagatggctatgacggtagctacttggaatgttacctgaaagatcataaaggtagctctgtggaaaatgcccgtgaagaagttattcggatgatttccgatgcttggaaacgcttgaatgaagaatgcttatttcccaaccccttttctgccacctttcgcaaagggtccttaaatattgctcgtatggtgcccctgatgtacagttacgatgacaaccataacctgcccattctggaagaacacatgaaaaccatgttgtatgattccagtagctaa

SEQ ID NO: 4 - protein, 590 aa, Coriandrum sativum
MAAITIFPLSYSIKFRRSSPCNPKDVTACKSVIKSVTGMTKVPVPVPEPIVRRSGNYKPCMWDNDFLQSLKTEYTGEAINARASEMKEEVRMIFNNVVEPLNQLELIDQLQRLGLDYHFRDEINHTLKNVHNGQKSETWEKDLHATALEFRLLRQHGHYISPEGFKRFTENGSFNKGIRADVRGLLSLYEASYFSIEGESLMEEAWSFTSNILKECLENTIDLDLQMQVRHALELPLQWRIPRFDAKWYINLYQRSGDMIPAVLEFAKLDFNIRQALNQEELKDLSRWWSRLDMGEKLPFARDRLVTSFFWSLGITGEPHHRYCREVLTKIIEFVGVYDDVYDVYGTLDELELFTNVVKRWDTNAMKELPDYMKLCFLSLINMVNETTYDILKDHNIDTLPHQRKWFNDLFERYIVEARWYNSGYQPTLEEYLKNGFVSIGGPIGVLYSYICTEDPIKKEDLEFIEDLPDIVRLTCEIFRLTDDYGTSSAELKRGDVPSSIYCYMSDTGVTEEVSRKHMMNLIRKKWAQINKLRFSKEYNNPLSWSFVDIMLNIIRAAHFLYNTGDDGFGVEDVAVEATLVSLLVEPIPL

SEQ ID NO: 5 - DNA, 1773 bp, Coriandrum sativum
atggcagcgataactatatttccactttcttattcgatcaaatttaggagatcctccccatgcaatcctaaagatgtgacagcctgcaagtctgtaattaaatccgtcactggaatgactaaggttcctgttccagtaccagagcctatcgtaaggcgatcagggaactacaaaccttgcatgtgggacaacgatttcttgcagtctttgaaaactgaatacaccggggaagcaatcaatgcacgagcttctgagatgaaggaagaggtgaggatgatatttaataatgtggtcgaaccattgaatcagcttgagctgattgatcagttgcagagacttgggttggattatcattttcgtgatgaaatcaaccatactttgaagaacgtacataatggtcagaagagtgagacttgggagaaggacttgcatgctactgctcttgaatttaggcttcttagacaacatggacattatatatcccctgagggcttcaagagatttacagagaatgggagcttcaataaaggtatccgtgcagatgtccggggactattaagtttatatgaagcctcgtacttttctattgaaggagagtccctgatggaggaggcttggtcctttacaagtaacatccttaaagagtgcctcgaaaatactattgatttggatctccagatgcaagtgagacatgctttggaacttccactacaatggaggatcccgagatttgatgcaaagtggtacataaatttgtatcaaagaagtggtgacatgatcccagcggttctggaatttgcaaagttggacttcaacattaggcaagcgttgaaccaagaagagcttaaagatttgtcgaggtggtggagtagattagacatgggagagaaacttccctttgccagagataggttggtaacatcatttttctggagtttggggattactggcgagcctcatcacagatattgcagagaggttttaaccaaaataatagagtttgttggtgtatacgatgatgtttatgatgtatatggtacacttgatgaacttgaactctttacaaatgtcgtgaagaggtgggatacaaatgcaatgaaagagctcccagactacatgaagttgtgcttcctgtcattgatcaacatggtcaatgaaacgacttacgacatcctcaaggaccataacatcgatactttaccacaccaaagaaaatggttcaatgatttattcgagcgttacatagtggaggcgaggtggtataacagtggataccagccaacactagaagaatacttgaaaaatggatttgtgtcaataggaggccccattggagtgctttactcttacatctgtactgaggatccaatcaagaaagaagatttagagtttatcgaggaccttcctgatatagtacgattgacatgtgaaatttttcggttaactgatgattatggaacatcttcggctgagttaaagagaggagatgttccatcttctatatattgctacatgtcggatactggtgttacggaagaagtttcccgtaagcacatgatgaacttgatcaggaagaagtgggcacaaattaacaaactcagattttcaaaggagtataataatcctttatcgtggtcttttgttgatattatgttgaatataatcagggcagcccattttttgtataatactggagacgatggctttggtgttgaagatgttgcagttgaagctacattagtttcgcttcttgtcgagcccattcctctctaa

SEQ ID NO: 6 - DNA, 1659 bp, Artificial Sequence
  DNA having modified codons, which encodes linalool synthase gene derived from Coriandrum sativum (opt_CsLINS)
atgactaaagtgcccgtgcccgtgcccgaacccattgtgcggcggagcggtaactataaaccctgtatgtgggataacgattttctgcaaagcttaaaaaccgaatatactggcgaagccattaatgcccgtgcttctgaaatgaaagaagaagtgcggatgatttttaacaacgtggttgaacccctgaaccaattggaactgattgatcaactgcagcgcctggggttggactaccattttcgtgatgaaattaaccataccttgaaaaacgtgcacaacggacaaaaatccgaaacctgggaaaaagatttacacgccactgctctggaatttcgtttgttacggcagcatggccactatattagccccgaaggttttaaacggtttaccgaaaatgggtcttttaacaaaggcattcgggccgatgtgcggggcctgttgtccctgtacgaagctagctacttttctattgaaggtgaaagtttgatggaagaagcctggtcctttactagtaacattttgaaagaatgtctggaaaacaccattgatttagacctgcaaatgcaggtgcgccatgccttggaattacccctgcaatggcgcattccccgttttgatgctaaatggtacattaacctgtaccagcgcagtggggacatgattcccgccgtgttggaatttgctaaactggattttaacattcgtcaagccttgaaccaggaagaattaaaagacctgagccgctggtggtctcgtctggatatgggcgaaaaattgccctttgctcgggatcgcttggtgacttcctttttctggagtttaggcattaccggtgaaccccatcaccggtactgtcgcgaagttctgaccaaaattattgaatttgtgggggtttacgatgacgtgtatgacgtttacggaaccttggatgaattggaactgtttactaacgtggttaaacgttgggacaccaacgccatgaaagaattacccgattatatgaaactgtgctttctgtccttgattaatatggtgaacgaaaccacttacgatattctgaaagaccataacattgataccttgccccaccaacgcaaatggtttaacgatctgtttgaacggtacattgtggaagcccgctggtataatagtggttaccagcccaccctggaagaatacttgaaaaatgggtttgtgtccattggcggtcccattggagttttgtacagttacatttgtactgaagaccccatcaaaaaagaagatttggaatttattgaagatttacccgacattgtgcgtctgacctgcgaaatttttcggctgaccgatgactatggcacttccagtgccgaattgaaacggggtgacgttcccagctctatttattgctacatgagcgataccggtgtgactgaagaagtttctcggaaacatatgatgaacctgattcgcaaaaaatgggcccaaattaacaaactgcggtttagcaaagaatataataaccccttgtcctggagttttgtggatattatgctgaacattattcgcgccgctcattttctgtacaacactggggatgacgggtttggagttgaagatgtggccgttgaagctaccttagtgagtttactggttgaacccattcccttataa

SEQ ID NO: 7 - DNA, 900 bp, Escherichia coli
atggactttccgcagcaactcgaagcctgcgttaagcaggccaaccaggcgctgagccgttttatcgccccactgccctttcagaacactcccgtggtcgaaaccatgcagtatggcgcattattaggtggtaagcgcctgcgacctttcctggtttatgccaccggtcatatgttcggcgttagcacaaacacgctggacgcacccgctgccgccgttgagtgtatccacgcttactcattaattcatgatgatttaccggcaatggatgatgacgatctgcgtcgcggtttgccaacctgccatgtgaagtttggcgaagcaaacgcgattctcgctggcgacgctttacaaacgctggcgttctcgattttaagcgatgccgatatgccggaagtgtcggaccgcgacagaatttcgatgatttctgaactggcgagcgccagtggtattgccggaatgtgcggtggtcaggcattagatttagacgcggaaggcaaacacgtacctctggacgcgcttgagcgtattcatcgtcataaaaccggcgcattgattcgcgccgccgttcgccttggtgcattaagcgccggagataaaggacgtcgtgctctgccggtactcgacaagtatgcagagagcatcggccttgccttccaggttcaggatgacatcctggatgtggtgggagatactgcaacgttgggaaaacgccagggtgccgaccagcaacttggtaaaagtacctaccctgcacttctgggtcttgagcaagcccggaagaaagcccgggatctgatcgacgatgcccgtcagtcgctgaaacaactggctgaacagtcactcgatacctcggcactggaagcgctagcggactacatcatccagcgtaataaataa

SEQ ID NO: 8 - DNA, 900 bp, Artificial Sequence
  DNA having modified codons, which encodes farnesyl diphosphate synthase gene derived from Escherichia coli (ispA gene)
atggattttccccagcagctggaagcctgcgtgaaacaggccaaccaggccctgagccgctttatcgcccccctgccctttcagaacacccccgtggtggaaaccatgcagtacggcgccctgctgggcggcaaacgcctgcgcccctttctggtgtacgccaccggccacatgtttggcgtgagcaccaacaccctggatgcccccgccgccgccgtggaatgcatccacgcctactttctgatccacgatgatctgcccgccatggatgatgatgatctgcgccgcggcctgcccacctgccacgtgaaatttggcgaagccaacgccatcctggccggcgatgccctgcagaccctggcctttagcatcctgagcgatgccgatatgcccgaagtgagcgatcgcgatcgcatcagcatgatcagcgaactggccagcgccagcggcatcgccggcatgtgcggcggccaggccctggatctggatgccgaaggcaaacacgtgcccctggatgccctggaacgcatccaccgccacaaaaccggcgccctgatccgcgccgccgtgcgcctgggcgccctgagcgccggcgataaaggccgccgcgccctgcccgtgctggataaatacgccgaaagcatcggcctggcctttcaggtgcaggatgatatcctggatgtggtgggcgataccgccaccctgggcaaacgccagggcgccgatcagcagctgggcaaaagcacctaccccgccctgctgggcctggaacaggcccgcaaaaaagcccgcgatctgatcgatgatgcccgccagagcctgaaacagctggccgaacagagcctggataccagcgccctggaagccctggccgattacatcatccagcgcaacaaatag

SEQ ID NO: 9 - DNA, 37 bp, Artificial Sequence
  Primer
acgttgttgccattgccctgttgacaattaatcatcg

SEQ ID NO: 10 - DNA, 37 bp, Artificial Sequence
  Primer
atgacttggttgagtttagctactggaatcatacaac

SEQ ID NO: 11 - DNA, 29 bp, Artificial Sequence
  Primer
tgtgaaattagctactggaatcatacaac

SEQ ID NO: 12 - DNA, 45 bp, Artificial Sequence
  Primer
gtagctaatttcacacaggagactgccatggattttccccagcag

SEQ ID NO: 13 - DNA, 37 bp, Artificial Sequence
  Primer
atgacttggttgagtctatttgttgcgctggatgatg

SEQ ID NO: 14 - DNA, 28 bp, Artificial Sequence
  Primer
tgtgaaattataagggaatgggttcaac

SEQ ID NO: 15 - DNA, 45 bp, Artificial Sequence
  Primer
ccttataatttcacacaggagactgccatggattttccccagcag

SEQ ID NO: 16 - DNA, 68 bp, Artificial Sequence
  Primer (gcd-attL)
ggtcaacattatggggaaaaactcctcatcctttagcgtgtgaagcctgcttttttatactaagttgg

SEQ ID NO: 17 - DNA, 68 bp, Artificial Sequence
  Primer (gcd-attR)
ttacttctggtcgggcagcgcataggcaatcacgtaatcgcgctcaagttagtataaaaaagctgaac

SEQ ID NO: 18 - DNA, 20 bp, Artificial Sequence
  Primer (gcd-t1)
tgacaacaatctatctgatt

SEQ ID NO: 19 - DNA, 20 bp, Artificial Sequence
  Primer (gcd-t2)
tgcgcctggttaagctggcg

SEQ ID NO: 20 - protein, 803 aa, Enterococcus faecalis
MKTVVIIDALRTPIGKYKGSLSQVSAVDLGTHVTTQLLKRHSTISEEIDQVIFGNVLQAGNGQNPARQIAINSGLSHEIPAMTVNEVCGSGMKAVILAKQLIQLGEAEVLIAGGIENMSQAPKLQRFNYETESYDAPFSSMMYDGLTDAFSGQAMGLTAENVAEKYHVTREEQDQFSVHSQLKAAQAQAEGIFADEIAPLEVSGTLVEKDEGIRPNSSVEKLGTLKTVFKEDGTVTAGNASTINDGASALIIASQEYAEAHGLPYLAIIRDSVEVGIDPAYMGISPIKAIQKLLARNQLTTEEIDLYEINEAFAATSIVVQRELALPEEKVNIYGGGISLGHAIGATGARLLTSLSYQLNQKEKKYGVASLCIGGGLGLAMLLERPQQKKNSRFYQMSPEERLASLLNEGQISADTKKEFENTALSSQIANHMIENQISETEVPMGVGLHLTVDETDYLVPMATEEPSVIAALSNGAKIAQGFKTVNQQRLMRGQIVFYDVADAESLIDELQVRETEIFQQAELSYPSIVKRGGGLRDLQYRAFDESFVSVDFLVDVKDAMGANIVNAMLEGVAELFREWFAEQKILFSILSNYATESVVTMKTAIPVSRLSKGSNGREIAEKIVLASRYASLDPYRAVTHNKGIMNGIEAVVLATGNDTRAVSASCHAFAVKEGRYQGLTSWTLDGEQLIGEISVPLALATVGGATKVLPKSQAAADLLAVTDAKELSRVVAAVGLAQNLAALRALVSEGIQKGHMALQARSLAMTVGATGKEVEAVAQQLKRQKTMNQDRALAILNDLRKQ

SEQ ID NO: 21 - DNA, 2412 bp, Enterococcus faecalis
atgaaaacagtagttattattgatgcattacgaacaccaattggaaaatataaaggcagcttaagtcaagtaagtgccgtagacttaggaacacatgttacaacacaacttttaaaaagacattccactatttctgaagaaattgatcaagtaatctttggaaatgttttacaagctggaaatggccaaaatcccgcacgacaaatagcaataaacagcggtttgtctcatgaaattcccgcaatgacggttaatgaggtctgcggatcaggaatgaaggccgttattttggcgaaacaattgattcaattaggagaagcggaagttttaattgctggcgggattgagaatatgtcccaagcacctaaattacaacgttttaattacgaaacagaaagctacgatgcgcctttttctagtatgatgtatgatggattaacggatgcctttagtggtcaggcaatgggcttaactgctgaaaatgtggccgaaaagtatcatgtaactagagaagagcaagatcaattttctgtacattcacaattaaaagcagctcaagcacaagcagaagggatattcgctgacgaaatagccccattagaagtatcaggaacgcttgtggagaaagatgaagggattcgccctaattcgagcgttgagaagctaggaacgcttaaaacagtttttaaagaagacggtactgtaacagcagggaatgcatcaaccattaatgatggggcttctgctttgattattgcttcacaagaatatgccgaagcacacggtcttccttatttagctattattcgagacagtgtggaagtcggtattgatccagcctatatgggaatttcgccgattaaagccattcaaaaactgttagcgcgcaatcaacttactacggaagaaattgatctgtatgaaatcaacgaagcatttgcagcaacttcaatcgtggtccaaagagaactggctttaccagaggaaaaggtcaacatttatggtggcggtatttcattaggtcatgcgattggtgccacaggtgctcgtttattaacgagtttaagttatcaattaaatcaaaaagaaaagaaatatggagtggcttctttatgtatcggcggtggcttaggactcgctatgctactagagagacctcagcaaaaaaaaaacagccgattttatcaaatgagtcctgaggaacgcctggcttctcttcttaatgaaggccagatttctgctgatacaaaaaaagaatttgaaaatacggctttatcttcgcagattgccaatcatatgattgaaaatcaaatcagtgaaacagaagtgccgatgggcgttggcttacatttaacagtggacgaaactgattatttggtaccaatggcgacagaagagccctcagttattgcggctttgagtaatggtgcaaaaatagcacaaggatttaaaacagtgaatcaacaacgcttaatgcgtggacaaatcgttttttacgatgttgcagatcccgagtcattgattgataaactacaagtaagagaagcggaagtttttcaacaagcagagttaagttatccatctatcgttaaacggggcggcggcttaagagatttgcaatatcgtacttttgatgaatcatttgtatctgtcgactttttagtagatgttaaggatgcaatgggggcaaatatcgttaacgctatgttggaaggtgtggccgagttgttccgtgaatggtttgcggagcaaaagattttattcagtattttaagtaattatgccacggagtcggttgttacgatgaaaacggctattccagtttcacgtttaagtaaggggagcaatggccgggaaattgctgaaaaaattgttttagcttcacgctatgcttcattagatccttatcgggcagtcacgcataacaaaggaatcatgaatggcattgaagctgtagttttagctacaggaaatgatacacgcgctgttagcgcttcttgtcatgcttttgcggtgaaggaaggtcgctaccaaggcttgactagttggacgctggatggcgaacaactaattggtgaaatttcagttccgcttgctttagccacggttggcggtgccacaaaagtcttacctaaatctcaagcagctgctgatttgttagcagtgacggatgcaaaagaactaagtcgagtagtagcggctgttggtttggcacaaaatttagcggcgttacgggccttagtctctgaaggaattcaaaaaggacacatggctctacaagcacgttctttagcgatgacggtcggagctactggtaaagaagttgaggcagtcgctcaacaattaaaacgtcaaaaaacgatgaaccaagaccgagccatggctattttaaatgatttaagaaaacaataa

SEQ ID NO: 22 - DNA, 2412 bp, Artificial Sequence
  DNA having modified codons, which encodes mvaE derived from Enterococcus faecalis
atgaaaaccgtggttattatcgatgcgctgcgcacgccgattggtaaatataaaggcagcctgtctcaagtgagcgccgttgatctgggtacgcatgtgaccacgcagctgctgaaacgtcacagcaccatctctgaagaaattgatcaggtgatctttggtaacgttctgcaagccggtaatggtcagaatccggcacgtcagattgcaatcaacagtggcctgagccatgaaattccggcgatgaccgtgaatgaagtttgcggtagcggcatgaaagcggttattctggccaaacagctgatccagctgggtgaagcggaagtgctgattgccggcggtatcgaaaacatgagtcaggcaccgaaactgcaacgttttaattatgaaaccgaaagctacgatgccccgttcagctctatgatgtatgatggcctgaccgatgcatttagcggtcaggcgatgggcctgacggcagaaaacgtggcggaaaaataccatgttacccgcgaagaacaggatcagttttctgttcacagtcagctgaaagcggcccaggcccaggcagaaggtattttcgccgatgaaatcgcaccgctggaagtgtctggtacgctggttgaaaaagatgaaggcattcgtccgaatagtagcgtggaaaaactgggcaccctgaaaacggtgttcaaagaagatggcaccgttacggcgggcaatgcaagcaccatcaatgatggtgcgagtgccctgattatcgcgagccaggaatatgcagaagcgcatggcctgccgtacctggccattatccgcgattctgtggaagttggtattgatccggcatatatgggcattagtccgatcaaagcgattcagaaactgctggcccgtaaccagctgaccaccgaagaaattgatctgtacgaaatcaatgaagcgtttgcagcgaccagtattgtggttcagcgcgaactggccctgccggaagaaaaagttaacatttatggcggtggcatcagcctgggtcacgcaattggtgccaccggtgcacgtctgctgaccagtctgagctatcagctgaatcagaaagagaaaaaatacggtgtggcaagcctgtgtattggtggcggtctgggtctggccatgctgctggaacgtccgcagcagaagaaaaactctcgtttttaccagatgagtccggaagaacgtctggccagtctgctgaacgaaggccagattagcgcagataccaaaaaagaattcgaaaatacggcactgtctagtcagatcgcgaaccatatgattgaaaatcagatcagcgaaaccgaagtgccgatgggtgttggcctgcacctgaccgtggatgaaacggattatctggttccgatggcgacggaagaaccgagcgttattgccgcactgtctaacggtgcaaaaatcgcgcagggctttaaaaccgtgaatcagcagcgtctgatgcgcggccagattgtgttctacgatgttgcggatccggaaagcctgatcgataaactgcaagtgcgcgaagccgaagtttttcagcaggcagaactgagctatccgtctattgtgaaacgtggcggtggcctgcgcgatctgcaataccgtacctttgatgaaagtttcgtgagcgttgatttcctggtggatgttaaagatgccatgggtgcaaacatcgtgaatgcgatgctggaaggcgttgccgaactgtttcgtgaatggttcgcggaacagaaaatcctgttttctatcctgagtaactacgcgaccgaaagcgtggttaccatgaaaacggccattcctgtgagccgcctgtctaaaggtagtaatggccgtgaaattgcggaaaaaatcgttctggcgagccgctatgcctctctggatccgtaccgtgccgtgacccataacaaaggtattatgaatggcatcgaagcagtggttctggcgaccggtaacgatacccgtgccgtgtctgcaagttgccatgcattcgcagttaaagaaggtcgttatcagggcctgaccagctggacgctggatggtgaacagctgatcggcgaaatttctgtgccgctggccctggcaaccgtgggtggcgcgacgaaagttctgccgaaaagccaggcggccgcagatctgctggcggtgaccgatgcaaaagaactgtctcgcgtggttgcggccgttggtctggcacagaatctggcagcgctgcgtgcgctggtgtctgaaggtattcagaaaggccacatggcactgcaagcccgtagtctggccatgaccgtgggtgcaacgggcaaagaagtggaagcagttgcgcagcagctgaaacgccagaaaaccatgaaccaggatcgtgccatggcaatcctgaatgatctgcgcaaacagtaa

SEQ ID NO: 23 - protein, 383 aa, Enterococcus faecalis
MTIGIDKISFFVPPYYIDMTALAEARNVDPGKFHIGIGQDQMAVNPISQDIVTFAANAAEAILTKEDKEAIDMVIVGTESSIDESKAAAVVLHRLMGIQPFARSFEIKEACYGATAGLQLAKNHVALHPDKKVLVVAADIAKYGLNSGGEPTQGAGAVAMLVASEPRILALKEDNVMLTQDIYDFWRPTGHPYPMVDGPLSNETYIQSFAQVWDEHKKRTGLDFADYDALAFHIPYTKMGKKALLAKISDQTEAEQERILARYEESIIYSRRVGNLYTGSLYLGLISLLENATTLTAGNQIGLFSYGSGAVAEFFTGELVAGYQNHLQKETHLALLDNRTELSIAEYEAMFAETLDTDIDQTLEDELKYSISAINNTVRSYRN

SEQ ID NO: 24 - DNA, 1152 bp, Enterococcus faecalis
atgacaattgggattgataaaattagtttttttgtgcccccttattatattgatatgacggcactggctgaagccagaaatgtagaccctggaaaatttcatattggtattgggcaagaccaaatggcggtgaacccaatcagccaagatattgtgacatttgcagccaatgccgcagaagcgatcttgaccaaagaagataaagaggccattgatatggtgattgtcgggactgagtccagtatcgatgagtcaaaagcggccgcagttgtcttacatcgtttaatggggattcaacctttcgctcgctctttcgaaatcaaggaagcttgttacggagcaacagcaggcttacagttagctaagaatcacgtagccttacatccagataaaaaagtcttggtcgtagcggcagatattgcaaaatatggcttaaattctggcggtgagcctacacaaggagctggggcggttgcaatgttagttgctagtgaaccgcgcattttggctttaaaagaggataatgtgatgctgacgcaagatatctatgacttttggcgtccaacaggccacccgtatcctatggtcgatggtcctttgtcaaacgaaacctacatccaatcttttgcccaagtctgggatgaacataaaaaacgaaccggtcttgattttgcagattatgatgctttagcgttccatattccttacacaaaaatgggcaaaaaagccttattagcaaaaatctccgaccaaactgaagcagaacaggaacgaattttagcccgttatgaagaaagtatcgtctatagtcgtcgcgtaggaaacttgtatacgggttcactttatctgggactcatttcccttttagaaaatgcaacgactttaaccgcaggcaatcaaattggtttattcagttatggttctggtgctgtcgctgaatttttcactggtgaattagtagctggttatcaaaatcatttacaaaaagaaactcatttagcactgctggataatcggacagaactttctatcgctgaatatgaagccatgtttgcagaaactttagacacagacattgatcaaacgttagaagatgaattaaaatatagtatttctgctattaataataccgttcgttcttatcgaaactaa

SEQ ID NO: 25 - DNA, 1152 bp, Artificial Sequence
  DNA having modified codons, which encodes mvaS derived from Enterococcus faecalis
atgaccattggtatcgataaaattagctttttcgtgccgccgtattacatcgatatgacggcgctggccgaagcacgtaacgttgatccgggcaaatttcatattggcatcggtcaggatcagatggcggtgaacccgatttctcaggatatcgttaccttcgcggccaatgcagcggaagcaattctgacgaaagaagataaagaagcgattgatatggtgatcgttggcaccgaaagctctatcgatgaaagtaaagccgcagcggtggttctgcaccgtctgatgggcattcagccgtttgcgcgcagcttcgaaatcaaagaagcctgctatggcgcgaccgccggtctgcaactggccaaaaaccatgtggcactgcacccggataaaaaagttctggtggttgccgcagatattgcgaaatacggtctgaatagcggcggtgaaccgacccagggtgcaggtgccgtggcaatgctggttgcatctgaaccgcgtattctggcgctgaaagaagataacgtgatgctgacccaggatatctatgatttttggcgtccgaccggtcatccgtacccgatggtggatggcccgctgagtaatgaaacctatattcagagcttcgcccaggtttgggatgaacataaaaaacgtacgggtctggattttgcggattatgatgcactggcgttccacattccgtacaccaaaatgggcaaaaaagcgctgctggccaaaatcagcgatcagacggaagccgaacaggaacgtattctggcacgctatgaagaaagcatcgtgtactctcgtcgcgttggcaacctgtataccggttctctgtacctgggcctgattagtctgctggaaaacgcgaccacgctgacggccggcaatcagatcggtctgttttcttatggcagtggtgccgtggcagaatttttcaccggtgaactggttgccggctaccagaaccatctgcaaaaagaaacccacctggccctgctggataatcgcacggaactgtctattgcagaatatgaagcaatgtttgcggaaaccctggatacggatatcgatcagaccctggaagatgaactgaaatatagtattagcgcgatcaacaatacggtgcgtagttaccgcaattaa

SEQ ID NO: 26 - DNA, 40 bp, Artificial Sequence
  Primer for amplifying a fragment comprising Para composed of araC and ara BAD promoters from E.coli
tgaattcgagctcggtacccactcttcctttttcaatatt

SEQ ID NO: 27 - DNA, 40 bp, Artificial Sequence
  Primer for amplifying a fragment comprising Para composed of araC and ara BAD promoters from E.coli
ataataaccacggttttcattttttataacctccttagag

SEQ ID NO: 28 - DNA, 40 bp, Artificial Sequence
  Primer for amplifying a fragment comprising EFmvaE gene
ctctaaggaggttataaaaaatgaaaaccgtggttattat

SEQ ID NO: 29 - DNA, 55 bp, Artificial Sequence
  Primer for amplifying a fragment comprising EFmvaE gene
ttatcgataccaatggtcatgtttttttacctcctttactgtttgcgcagatcat

SEQ ID NO: 30 - DNA, 55 bp, Artificial Sequence
  Primer for amplifying a fragment comprising EFmvaS gene
atgatctgcgcaaacagtaaaggaggtaaaaaaacatgaccattggtatcgataa

SEQ ID NO: 31 - DNA, 40 bp, Artificial Sequence
  Primer for amplifying a fragment comprising EFmvaS gene
cagcggaactggcggctcccttaattgcggtaactacgca

SEQ ID NO: 32 - DNA, 40 bp, Artificial Sequence
  Primer for amplifying a fragment comprising Ttrp
tgcgtagttaccgcaattaagggagccgccagttccgctg

SEQ ID NO: 33 - DNA, 38 bp, Artificial Sequence
  Primer for amplifying a fragment comprising Ttrp
gtcgactctagaggatccctaatgagaattagtcaaat

SEQ ID NO: 34 - DNA, 42 bp, Artificial Sequence
  Primer (Linker-F)
agctttagggataacagggtaatctcgagctgcaggcatgca

SEQ ID NO: 35 - DNA, 42 bp, Artificial Sequence
  Primer (Linker-R)
agcttgcatgcctgcagctcgagattaccctgttatccctaa

SEQ ID NO: 36 - DNA, 55 bp, Artificial Sequence
  Primer (lldD5' CAS)
tttttaagctttagggataacagggtaatctcgagatttaaagcggctgctttac

SEQ ID NO: 37 - DNA, 43 bp, Artificial Sequence
  Primer (lldD3' CAS)
tttttaagcttgcatgcctgcagtatttaatagaatcaggtag

SEQ ID NO: 38 - DNA, 54 bp, Artificial Sequence
  Primer (phoC5' CAS)
tttttaagctttagggataacagggtaatctcgagtggataacctcatgtaaac

SEQ ID NO: 39 - DNA, 44 bp, Artificial Sequence
  Primer (phoC3' CAS)
tttttaagcttgcatgcctgcagttgatgtctgattatctctga

SEQ ID NO: 40 - DNA, 54 bp, Artificial Sequence
  Primer (pstS5' CAS)
tttttaagctttagggataacagggtaatctcgagagcctctcacgcgtgaatc

SEQ ID NO: 41 - DNA, 44 bp, Artificial Sequence
  Primer (pstS3' CAS)
tttttaagcttgcatgcctgcagaggggagaaaagtcaggctaa

SEQ ID NO: 42 - DNA, 33 bp, Artificial Sequence
  Primer (n67)
tgcgaagacgtcctcgtgaagaaggtgttgctg

SEQ ID NO: 43 - DNA, 36 bp, Artificial Sequence
  Primer (n68)
tgcgaagggccccgttgtgtctcaaaatctctgatg

SEQ ID NO: 44 - DNA, 70 bp, Artificial Sequence
  Primer (ampH-attL-phi80)
atgcgcactccttacgtactggctctactggtttctttgcgaaaggtcatttttcctgaatatgctcaca

SEQ ID NO: 45 - DNA, 64 bp, Artificial Sequence
  Primer (ampH-attR-phi80)
ttaaggaatcgcctggaccatcatcggcgagccgttctgacgtttgttgacagctggtccaatg

SEQ ID NO: 46 - DNA, 68 bp, Artificial Sequence
  Primer (DampC-phL)
ctgatgaactgtcacctgaatgagtgctgatgaaaatatagaaaggtcatttttcctgaatatgctca

SEQ ID NO: 47 - DNA, 64 bp, Artificial Sequence
  Primer (DampC-phR)
attcgccagcataacgatgccgctgttgagctgaggaacacgtttgttgacagctggtccaatg

SEQ ID NO: 48 - DNA, 18 bp, Artificial Sequence
  Primer (ampH-t1)
gcgaagccctctccgttg

SEQ ID NO: 49 - DNA, 21 bp, Artificial Sequence
  Primer (ampH-t2)
agccagtcagcctcatcagcg

SEQ ID NO: 50 - DNA, 21 bp, Artificial Sequence
  Primer (ampC-t1)
gattcccacttcaccgagccg

SEQ ID NO: 51 - DNA, 21 bp, Artificial Sequence
  Primer (ampC-t2)
ggcaggtatggtgctctgacg

SEQ ID NO: 52 - DNA, 64 bp, Artificial Sequence
  Primer (crtE-attRphi80)
atgacggtctgcgcaaaaaaacacgttcatctcactcgcgcgtttgttgacagctggtccaatg

SEQ ID NO: 53 - DNA, 68 bp, Artificial Sequence
  Primer (crtZ-attLphi80)
atgttgtggatttggaatgccctgatcgttttcgttaccggaaaggtcatttttcctgaatatgctca

SEQ ID NO: 54 - DNA, 21 bp, Artificial Sequence
  Primer (crtZ-test)
ccgtgtggttctgaaagccga

SEQ ID NO: 55 - DNA, 21 bp, Artificial Sequence
  Primer (crtE-test)
cgttgccgtaaatgtatccgt

SEQ ID NO: 56 - DNA, 27 bp, Artificial Sequence
  Primer (phL-test)
ggatgtaaaccataacactctgcgaac

SEQ ID NO: 57 - DNA, 25 bp, Artificial Sequence
  Primer (phR-test)
gattggtggttgaattgtccgtaac

SEQ ID NO: 58 - DNA, 3471 bp, Artificial Sequence
  Sequence of the chemically synthesized DNA fragment retaining artificial KDyI operon with optimized codons
gcatgcaggaggtatgaatgtcagagttgcgtgccttcagtgccccagggaaagcgttactcgctggtggatatttagttttagatacaaaatatgaagcatttgtagtcggattatcggcacgtatgcacgctgtagcccatccttacggttcattgcaagggtctgataagtttgaagtgcgtgtgaaaagtaaacaatttaaagatggggagtggctgtaccatataagtcctaaaagtggcttcattcctgtttcgataggcggatctaagaaccctttcattgaaaaagttatcgctaacgtatttagctactttaaacctaacatggacgactactgcaatcgtaacttgttcgttattgatattttctctgatgatgcctaccattctcaggaggatagcgttaccgaacatcgtggcaaccgccgtttgagttttcattcgcaccgtattgaagaagttcccaaaacagggctgggctcctcggcaggtttagtcacagttttaactacagctttggcctccttttttgtatcggacctggaaaataatgtagacaaatatcgtgaagttattcataatttagcacaagttgctcattgtcaagctcagggtaaaattggaagcgggtttgatgtagcggcggcagcatatggatctatccgttatcgccgtttcccacccgcattaatctctaatttgccagatattggaagtgctacttacggcagtaaactggcgcatttggttgatgaagaagactggaatattacgattaaaagtaaccatttaccttcgggattaactttatggatgggcgatattaagaatggttcagaaacagtaaaactggtccagaaggtaaaaaattggtatgattcgcatatgccagaaagcctcaaaatatatacagaactcgatcatgcaaattctcgttttatggatggactctctaaactcgatcgcttacacgagactcatgacgattacagcgatcagatatttgagtctcttgagcgtaatgactgtacctgtcaaaagtatcctgaaatcacagaagttcgtgatgcagttgccacaattcgtcgttcctttcgtaaaataactaaagaatctggtgccgatatcgaacctcccgtacaaactagcttattggatgattgccagaccttaaaaggagttcttacttgcttaatacctggtgctggtggttatgacgccattgcagtgattactaagcaagatgttgatcttcgtgctcaaaccgctaatgacaaacgtttttctaaggttcaatggctggatgtaactcaggctgactggggtgttcgtaaagaaaaagatccggaaacttatcttgataaataactgcagaggaggtatgaatgaccgtttacacagcatccgttaccgcacccgtcaacatcgcaacccttaagtattgggggaaacgtgacacgaagttgaatctgcccaccaattcgtccatatcagtgactttatcgcaagatgacctccgtacgttgacctctgcggctactgcacctgagtttgaacgcgacactttgtggttaaatggagaaccacacagcatcgacaatgaacgtactcaaaattgtctgcgcgacctccgccaattacgtaaggaaatggaatcgaaggacgcctcattgcccacattatctcaatggaaactccacattgtctccgaaaataactttcctacagcagctggtttagcttcctccgctgctggctttgctgcattggtctctgcaattgctaagttataccaattaccacagtcaacttcagaaatatctcgtatagcacgtaaggggtctggttcagcttgtcgttcgttgtttggcggatacgtggcctgggaaatgggaaaagctgaagatggtcatgattccatggcagtacaaatcgcagacagctctgactggcctcagatgaaagcatgtgtccttgttgtcagcgatattaaaaaggatgtgagttccactcagggtatgcaattgaccgtggcaacctccgaactctttaaagaacgtattgaacatgtcgtaccaaagcgttttgaagtcatgcgtaaagccattgttgaaaaagatttcgccacctttgcaaaggaaacaatgatggattccaactctttccatgccacatgtttggactctttccctccaatattctacatgaatgacacttccaagcgtatcatcagttggtgccacaccattaatcagttttacggagaaacaatcgttgcatacacgtttgatgcaggtccaaatgctgtgttgtactacttagctgaaaatgagtcgaaactctttgcatttatctataaattgtttggctctgttcctggatgggacaagaaatttactactgagcagcttgaggctttcaaccatcaatttgaatcatctaactttactgcacgtgaattggatcttgagttgcaaaaggatgttgcccgtgtgattttaactcaagtcggttcaggcccacaagaaacaaacgaatctttgattgacgcaaagactggtctcccaaaggaataaggatccaggaggtatgaatgactgccgacaacaatagtatgccccatggtgcagtatctagttacgccaaattagtgcaaaaccaaacacctgaagacattttggaagagtttcctgaaattattccattacaacaacgtcctaatacccgctctagtgagacgtcaaatgacgaaagcggagaaacatgtttttctggtcatgatgaggagcaaattaagttaatgaatgaaaattgtattgttttggattgggacgataatgctattggtgccggcaccaagaaagtttgtcatttaatggaaaatattgaaaagggtttacttcatcgtgcattctccgtctttattttcaatgaacaaggtgaattacttttacaacaacgtgccactgaaaaaataactttccctgatctttggactaacacatgctgctctcatccactttgtattgatgacgaattaggtttgaagggtaagctcgacgataagattaagggcgctattactgcggcggtgcgtaaactcgatcatgaattaggtattccagaagatgaaactaagacacgtggtaagtttcactttttaaaccgtatccattacatggcaccaagcaatgaaccatggggtgaacatgaaattgattacatcctcttttataagatcaacgctaaagaaaacttgactgtcaacccaaacgtcaatgaagttcgtgacttcaaatgggtttcaccaaatgatttgaaaactatgtttgctgacccaagttacaagtttacgccttggtttaagattatttgcgagaattacttattcaactggtgggagcaattagatgacctttctgaagtggaaaatgaccgtcaaattcatcgtatgctctaaggtacc

SEQ ID NO: 59 - DNA, 2931 bp, Pantoea anantis
  CDS (301)..(2691)
gcgtctggcgatctcattccctttacgctttaacctttcttatctcctggcactattgaatcatatcggcaaggccccattaacaccctctaaagtattgccttagatgcgttgttaagagctttaagccaaaaaaatcaaaactcataccaattttgctataacatttaacagatatggatcatcacgcttcagggaagagcgaaataagaatgcctttcatcttttgtactttatgactgacaacaatctatctgattgttttcctgagttttctggcaacgaaatgaggtcaacattatggggaaaaactcctcatcctttagcgtggtccgttttttaacggtgctgttcgccgtgctaacgggtgcgttcatgttaattggtggtatctggctggccacgatcggtggttcctggtactacatcatcggcggtgcagccatgctgcttaccgctttcctgctgtggcgacgtaacagcgctgccctggttgtctatgcgctcttactgctggctacgctggcctggggcgtttgggaagtcggcaccgacttctgggcactggcaccgcgtaccgacgtactggtgatctttggcgtctggctggtgttgccctttgtctatcgcggcttataccagccgggtaaaggcgcactgggtgccatgggcgtagcgctggttgccagtgcagcggtgttaacctattccgtctttaatgatccgcaagtggttaacggtgcattaccggcaacagcggataatgcgcctcaggcacagccgttgagcaatattgctgatggtgactggccggcctatgcgcgcgatcagcaagggacgcgcttctcgccgctcaagcagatcaaccacgacaatgtgaaagaactgcaggttgcctggcaattccagaccggtgatatgaaacgcccaagcgatccgggcgaaattaccgatgaagtgacgccaatcaagattcgcgacacgctgtatctttgcacgccacatcagattttatttgctctggatgcggccaccggcaagcaaaagtggaagtttgatcccggcctgaaaaccaacccaaccttccagcacgtgacctgtcgtggtgtgtcataccacgaattccctgcagcgaaggatgcgtccaatacccagcctgcgctgtgctcgcgtcgtatctacctgccagtcaatgacgggcgtttgttcgcgctggatgcggaaaccggtgaacgctgcccggcctttggtaacaacggtgagctggatctgcagcacaagcagccggtcacaacgccaggcatgtatgagccaacctcgccaccggtgattactgacaccaccattgtgatggctggcgcggtaaccgataacttttcaacccgtgaaccttcaggcgccatccgtggctttgatgtgaacaccggtaagctgttgtgggtgttcgatccgggcgcgaaagatcctaacgcgattccggcggatgaacacacgttcaccatgaactcccctaactcgtgggcacctgcggtttacgatccgaagctggatatcgtttacctgccaatgggggtgaccacgccggatatctggggcggcaaccgcacacctgagcaggaacgttatgccagcagcgtgctggcgctgaacgcgacgaccggtaagctggtgtggtcatatcagactgtgcatcacgatctgtgggatatggacctgccttcgcagccgacgctggcggatattaccgataaagacggtaataccgtgccggttatctatgcccctgccaaaaccgggaacatctttgttctggatcgccgcacaggtaaaactgtggttccggccccggaaacccctgttccgcagggcgcagctaagggcgaccatgtctcagctacacagccttactctgaactgaccttccgtccgaaacagaacctgacggataaggacatgtggggcgcgacgatgtatgaccagctggtgtgccgcgtgattttcaaacgtctgcgctacgaaggtccgttcacgccaccttctgagcagggcaccctggtcttcccgggcaacctgggcatgtttgaatggggcggcatttccgttgatccgcatcgtcagattgcgattgctaacccaatggcgctgccgttcgtgtctaagctgatcccacgcggtccgggtaatccggaagagccaccaaaaggcgcaacgggcggttcaggtactgaaaccggtattcagccgcagtacggtgtgccatatggcgttgaactgaatccgttcctgtcaccttttggtctgccgtgtaaacaacctgcatggggttatgtttctgctgttgacctgaaaaccaacgaagtggtgtggaaacaacgtattggtaccgttcgtgacagctcacctgtaccgctgccctttaaaatgggtatgccaatgctgggcggaccggttgccaccgcaggcaaagtgttctttattggcgcaacggctgataactacctgcgcgctttcagcaccgacaccggtgaactcttgtggcaggcgcgcctgccagccggtggtcaggcaacgccaatgacctatgaagttaacggcaagcaatacgttgtgattgctgccggtggccatggttcattcggcaccaagctgggcgattacgtgattgcctatgcgctgcccgaccagaagtaattaacacctgaacagaggcggactccggtccgcctttttttatgcctgctatctgccctgtgcttttgcgcgtggggagcgccagcttaaccaggcgcacagccccatgaccatgcaggtggccagaaatactggccgcattccccacgcgccaccaatcaccccaccaaaaaggggaccactgacctggccgatatactgcgccgacgtcgaatagccgagcatgcgccccacctgcac

SEQ ID NO: 60 - protein, 796 aa, Pantoea anantis
MGKNSSSFSVVRFLTVLFAVLTGAFMLIGGIWLATIGGSWYYIIGGAAMLLTAFLLWRRNSAALVVYALLLLATLAWGVWEVGTDFWALAPRTDVLVIFGVWLVLPFVYRGLYQPGKGALGAMGVALVASAAVLTYSVFNDPQVVNGALPATADNAPQAQPLSNIADGDWPAYARDQQGTRFSPLKQINHDNVKELQVAWQFQTGDMKRPSDPGEITDEVTPIKIRDTLYLCTPHQILFALDAATGKQKWKFDPGLKTNPTFQHVTCRGVSYHEFPAAKDASNTQPALCSRRIYLPVNDGRLFALDAETGERCPAFGNNGELDLQHKQPVTTPGMYEPTSPPVITDTTIVMAGAVTDNFSTREPSGAIRGFDVNTGKLLWVFDPGAKDPNAIPADEHTFTMNSPNSWAPAVYDPKLDIVYLPMGVTTPDIWGGNRTPEQERYASSVLALNATTGKLVWSYQTVHHDLWDMDLPSQPTLADITDKDGNTVPVIYAPAKTGNIFVLDRRTGKTVVPAPETPVPQGAAKGDHVSATQPYSELTFRPKQNLTDKDMWGATMYDQLVCRVIFKRLRYEGPFTPPSEQGTLVFPGNLGMFEWGGISVDPHRQIAIANPMALPFVSKLIPRGPGNPEEPPKGATGGSGTETGIQPQYGVPYGVELNPFLSPFGLPCKQPAWGYVSAVDLKTNEVVWKQRIGTVRDSSPVPLPFKMGMPMLGGPVATAGKVFFIGATADNYLRAFSTDTGELLWQARLPAGGQATPMTYEVNGKQYVVIAAGGHGSFGTKLGDYVIAYALPDQK

SEQ ID NO: 61 - protein, 333 aa, Streptomyces clavuligerus
MGSLMQEFEFAVPAPSRVSPDLARARARHLDWVHAMDLVRGEEARRRYEFSCVADIGAYGYPHATGADLDLCVDVLGWTFLFDDQFDAGDGRERDALAVCAELTDLLWKGTAATAASPPIVVAFSDCWERMRAGMSDAWRRRTVHEWVDYLAGWPTKLADRAHGAVLDPAAHLRARHRTICCRPLFALAERVGGYEVPRRAWHSSRLDGMRFTTSDAVIGMNELHSFEKDRAQGHANLVLSLVHHGGLTGPEAVTRVCDLVQGSIESFLRLRSGLPELGRALGVEGAVLDRYADALSAFCRGYHDWGRGASRYTTRDHPGDLGLENLVARSSG

SEQ ID NO: 62 - DNA, 1002 bp, Streptomyces clavuligerus
ttggggtcattgatgcaggaattcgaattcgcggtgcccgcgccgagccgtgtcagtccggatctcgcccgcgcgagggcccgtcatctcgactgggtccacgccatggacctggtgcgcggcgaggaggccaggcggcgttacgagttctcctgtgtggccgacatcggcgcctatggatatccgcacgcgaccggtgcggacctggatctctgcgtcgacgtcctcgggtggaccttcctcttcgacgatcaattcgacgccggggacgggcgggagcgggacgctttggcggtctgcgcggagctgacggacctgttgtggaaggggacggcggccacggcggcctcgccgccgatcgtggtggcgttcagcgactgctgggagcggatgcgggcgggcatgtcggacgcgtggcggcggcggacggtccatgagtgggtggactatctggcgggctggcccaccaagctcgccgaccgcgcgcacggcgccgtcctggacccggccgcgcatctgcgcgcgcggcaccggacgatctgctgccgcccgctcttcgccctggcggaacgggtcggggggtacgaggtcccgcggcgggcctggcactccagccggctcgacgggatgcggttcaccacgtccgatgcggtgatcggcatgaacgagctccactcgttcgagaaggaccgggcgcagggccacgccaacctcgtcctgagcctcgtgcaccacggcggactcaccgggccggaggccgtcacccgggtgtgcgacctggtccagggctcgatcgagtccttcctgcgactgcggtccgggctgccggagctgggccgggccctcggtgtcgagggggccgtgctcgaccggtacgccgacgcgctgtccgcgttctgccgcgggtaccacgactggggtcgcggcgcctcgcggtacaccacccgcgatcaccccggcgatctcggactggagaatctcgtcgcccggtcgtcgggctga

SEQ ID NO: 63 - DNA, 1002 bp, Artificial Sequence
  DNA having modified codons, which encodes linalool synthase gene derived from Streptomyces clavuligerus (opt_ScLINS)
atgggttctctgatgcaggaatttgaatttgctgtgcccgctccctctcgcgttagccccgatttagcccgtgctcgtgctcgtcatctggattgggttcatgccatggacttagttcggggtgaagaagcccggcgccgttatgaatttagctgtgtggctgatattggcgcctatggttacccccatgccaccggcgctgatctggacttgtgcgtggatgttttgggttggacctttttatttgatgaccaatttgatgctggagacggtcgtgaacgtgatgctctggctgtgtgtgccgaattgaccgacttgttatggaaaggaaccgctgctactgctgctagcccccccattgtggttgccttttctgattgctgggaacggatgcgggctggtatgagtgacgcttggcggcgccgtaccgtgcatgaatgggttgattatttggccgggtggcccactaaattagccgatcgtgctcacggagctgtgttagaccccgctgctcatctgcgtgctcgtcaccgtaccatttgttgccgccccctgtttgccttggctgaacgtgtgggaggttacgaagttccccgtcgtgcttggcattccagtcgtttggatggtatgcggtttaccacttccgacgccgtgattggtatgaacgaactgcatagttttgaaaaagatcgtgctcaagggcacgccaacttagtgctgtccttggttcatcacggaggattgaccggacccgaagctgtgactcgtgtttgtgatttagttcagggctccattgaatcctttttgcggctgcgcagtgggttacccgaactgggacgtgctctgggagtggaaggagctgttttggatcggtacgccgacgctttaagcgctttttgccgcgggtatcatgattgggggcgtggagcctctcggtacaccactcgcgatcaccccggcgacttgggtttagaaaatttggtggcccgcagctctggctaa

SEQ ID NO: 64 - DNA, 30 bp, Artificial Sequence
  Primer
gtgtgaaattagccagagctgcgggccacc

SEQ ID NO: 65 - DNA, 44 bp, Artificial Sequence
  Primer
tggctaatttcacacaggagactgccatggattttccccagcag

SEQ ID NO: 66 - DNA, 33 bp, Artificial Sequence
  Primer
atgacttggttgagtttagccagagctgcgggc

SEQ ID NO: 67 - DNA, 37 bp, Artificial Sequence
  Primer
acgttgttgccattgccctgtttgcaattaatcatcg

SEQ ID NO: 68 - DNA, 36 bp, Artificial Sequence
  Primer
atgacttggttgagtttataagggaatgggttcaac

SEQ ID NO: 69 - protein, 567 aa, Artemisia annua
GNAYMRIYSTKTTRITANATVNAADTHVRRSANYKPSSWSFDHIQSLSSKYTGDDYVARANTLKDAVKTMIRKSGNSLRTLELVDELQRLGISYLFEEEISNLLETIYYNYYKFPENWNKINLNLKALGFRLLRQHGYHVPQEIFLNFKDKNQNLNSYLLNDVVEMLNLYEASYHSFEDESILDDARDITTKYLKESLEKIDGSIFSSVTHALEQPLHWRVPRVEAKWFIELYEKKNGMSPTLVELAKLDFDMVQAIHLEDLKHASRWWRDTSWDTKLTFARDLIVENFLWTIGFSYLPNFSRGRRTITKVAVMITTLDDVYDVFGTLGELEQFTDVINRWDIKAIEQLPDYMKICFLGLYKSINDITHETLANKGFLILPYLKKAWADLCKAYLVEAQWYHRGHIPTLNEYLDNACVSISGPVALMHVHFLTSVSSIEEIHQCIQRTENIVHYVSLIFRLADDLGTSLGEMERGDTLKSIQLHMHETGATEPEARSYIKLLINKTWKKLNKERATVNSESSQEFIDYATNLVRMAQFMYGEGDEDFGLDVIKSHVLSLLFTPIQGI

SEQ ID NO: 70 - DNA, 1704 bp, Artemisia annua
ggtaatgcttacatgcgaatatattcaacaaaaaccacaagaataactgccaatgcaactgtcaatgcagctgacacccacgtaaggcgatcagcaaattacaaaccatcatcatggtcatttgatcatattcagtcactctctagtaaatacacgggagatgattacgtggcaagagcaaatactttgaaggacgcagtgaagacgatgatacgaaaatcaggaaattcgttgagaactctggagctagttgatgagttgcaaagattaggaatctcgtatctttttgaggaggaaataagtaatctcttggaaacgatttactacaattactataaatttcctgaaaattggaataagatcaatttgaaccttaaggctcttggctttcgattactgagacaacatggttatcatgttcctcaagagatatttctcaactttaaggacaagaatcaaaatcttaattcatatttactcaacgatgttgtggaaatgctcaacctgtatgaggcatcttatcattcgttcgaggatgaaagcatattggacgacgctagagacatcacaaccaaatatctcaaagaaagcttggagaagattgacgggagtatcttttcatcagtaactcatgctttggagcaaccgctgcattggagggtaccgagagttgaggcgaagtggtttattgaactatatgagaaaaagaatggcatgagtcccacattagtcgagcttgcgaaattggatttcgatatggtccaggctatccatcttgaggatctaaaacacgcatcaaggtggtggagagatacaagttgggataccaagttaacctttgcaagggacttgatagtggagaatttcttgtggacaattggtttcagttacttaccaaactttagtcgtgggaggagaacaataactaaggtggccgttatgattactactctcgatgatgtctatgatgtgtttggtactttgggcgaactagaacaattcactgatgttataaacagatgggatataaaggcgattgaacaactcccagattatatgaagatatgtttcttaggactttacaagtcgataaatgatatcacgcatgaaactttggcaaacaaaggattcctcattcttccatatttaaagaaagcatgggcagatctatgtaaggcgtacctagtagaagctcaatggtaccaccgtggacatataccaacactgaacgagtacttggacaatgcttgtgtatcgatatcaggacctgtagcacttatgcatgtccactttttaacatcagttagttcaatcgaagaaatccatcaatgcatacaaagaactgagaatatagttcactatgtatcacttatcttccgacttgctgatgacttggggacatcattaggtgaaatggaaagaggtgatactctaaaatcaatccagttgcacatgcatgagaccggtgctactgaaccagaagctagaagttatataaaattgttaatcaacaaaacatggaagaaacttaacaaagaacgagcaactgttaactccgaatcttcacaggagtttattgattatgcaacaaaccttgttagaatggctcaattcatgtacggtgaaggagacgaggattttggtctagatgtgattaaatctcatgtattatcattgttgtttactccaatccaagggatataa

SEQ ID NO: 71 - DNA, 1623 bp, Artificial Sequence
  DNA having modified codons, which encodes linalool synthase gene derived from Artemisia annua (opt_AnLINS)
atgcggcggagtgctaactacaaaccctcttcttggtcctttgatcacattcagtccctgtccagtaaatacaccggagacgattatgtggcccgcgctaataccttgaaagatgccgttaaaactatgattcgtaaatccggcaatagtttacggaccttagaactggtggacgaactgcaacgtttgggtatttcctatttgtttgaagaagaaattagtaacttgctggaaaccatttactacaactactacaaatttcccgaaaactggaacaaaattaacttgaacctgaaagccttagggtttcgtctgttgcggcaacatggatatcacgtgccccaggaaatttttctgaactttaaagataaaaaccagaacttgaatagttacttactgaacgacgtggttgaaatgctgaatttgtatgaagctagctaccattcttttgaagatgaatccattttggatgacgcccgggacattaccactaaatacctgaaagaatccttggaaaaaattgatggcagtatttttagtagtgtgacccatgctttagaacaacccctgcactggcgcgtgccccgtgttgaagccaaatggtttattgaactgtacgaaaagaaaaatggcatgagtcccaccttagtggaactggccaaattggattttgacatggttcaggctattcatttagaagatctgaaacacgccagccggtggtggcgcgatacctcttgggacaccaaattaacttttgcccgtgatctgattgtggaaaattttctgtggaccattggctttagctatttgcccaacttttctcggggtcggcgcaccattactaaagtggccgttatgattaccactttagatgacgtgtacgatgtttttgggaccttgggagaactggaacaatttactgatgtgattaatcgttgggacattaaagctattgaacagttgcccgattatatgaaaatttgttttctggggctgtacaaaagtattaacgacattacccatgaaactctggccaacaaaggatttttgattctgccctacctgaaaaaagcctgggctgatttgtgtaaagcctatttagtggaagctcaatggtaccatcgcggtcacattcccaccttgaacgaatacttagataatgcttgcgtgagcatttctgggcccgtggccttaatgcatgttcactttctgacctccgttagctctattgaagaaattcatcaatgcattcagcgcactgaaaatattgtgcactatgttagcctgatttttcgtttggccgatgacttaggcacctctctgggtgaaatggaacggggggatactctgaaatccattcaattgcatatgcacgaaaccggagccactgaacccgaagctcggagttacattaaattgctgattaacaaaacctggaaaaaattgaataaagaacgcgccactgtgaacagcgaatccagtcaagaatttattgattacgccaccaacttagttcgcatggctcagtttatgtacggcgaaggtgatgaagactttggcttggatgtgattaaatcccatgttctgagtctgttgtttacccccattcaaggtatttaa

SEQ ID NO: 72 - protein, 594 aa, Backhousia citriodora
MALPALFGSSLPSSIRHNQPSLFSFRHPRFCSSSSSASFSSQFILCASKTGDQEIVRRSANWQPSVWDYDYVQSLTVDYTEDKYTKQVQRLKEEVKGLFDREMKQVAKLEFIDVVQRLGLGYHFKTEIKIALSSIHNNTEDAQLSNDLYAASLRFRLLRQYGCNVQQDVFQRFMNKTGTFKESLNKDVKGILGLYEASFHGMEGETVLDEAWNFASKHLKDLNLDEVPTNLASNVSHALDMPIHWRPNRLEARWFMDMYEKQQDLIPSLLRLAKLDFNIVQSIHRKEVSNLARWWVELGANKMTFFRDRLVESYFWSCILVFEPQYTDFRELNTRIACMATLIDDVYDIYGTPEELELLTDFILRWDITDIDKLPPTIRNGFMALYNTTNKVGYRTMTKRGINPIPYLRKLWGDECKADMKEVHWFNNGIKPTLKEYMDVAVDSIGGLILLLNSYFLTTDYLTEEGLNYVSKIPSVMHSSAQIFRFNDDLSTSSHELARGDNSKALECYMNETGASEEIAREHIRHLVRETWKKMNKEVFEDYPFSGFGPFLSACLNLARASHCFYEYGDGYGLPDHQTRDHLASTIFESVSLD

SEQ ID NO: 73 - DNA, 1785 bp, Backhousia citriodora
atggctcttcctgctctttttggaagctccctcccctcctcaatccgccataaccaaccctctctcttttcctttagacaccctcgcttctgctcctcctcctcttccgcctccttcagcagccagtttattttatgcgcttcgaagactggggatcaagagattgtgagacgttccgcgaattggcaacctagcgtctgggactacgactatgtgcagtcacttactgttgattacacggaggataaatataccaaacaagtccaaaggttaaaggaagaagtcaagggtttattcgatagggagatgaaacaggtagccaagctcgagttcatagatgtggttcaaagactaggacttggataccatttcaagaccgagataaaaattgctctcagttccattcataacaacaccgaagatgcgcaactttcgaatgatctctatgctgcttcccttcgattccgactactcagacaatatggatgtaacgtgcagcaagatgtgtttcaaaggtttatgaacaagacgggcacattcaaggaatcactcaataaggatgtgaaggggattcttggtctttatgaagcttcttttcacggaatggaaggtgaaaccgtactcgatgaagcttggaactttgcttctaagcatctgaaggatctaaacctcgacgaagttcccaccaatttggcgagcaacgtgagtcatgcattagacatgccgattcattggaggccaaacagactagaggctcggtggttcatggacatgtacgagaaacagcaagacttgatcccctctttgctgcgattggctaaattagacttcaatatagtgcagtcgatccacaggaaggaagttagcaatcttgcaaggtggtgggttgaacttggggcgaacaagatgaccttctttagggacaggctggtggaaagctatttttggagttgtatacttgttttcgaacctcaatatacagatttcagagaactaaatacaaggattgcttgcatggcgacacttatcgatgatgtttacgatatatatgggactccggaagagcttgaactcttaacagatttcattctcaggtgggacatcacagatatcgataagcttcctccaacaataaggaacggtttcatggccttatacaacacgaccaacaaagttgggtatcggacgatgacaaagcgaggaatcaatcccatcccttacttgcgtaaattgtggggcgatgaatgcaaggcggacatgaaggaggtccattggttcaataatggcattaaaccgacgctgaaggagtacatggacgttgcggtggattcaatcggagggctgattttgctgttgaatagctacttcctaaccacagactatttgacggaagagggacttaattacgtgtcgaaaatcccaagtgtcatgcattcttctgcccagatctttcgattcaacgatgatctcagtacatcatcgcatgaattggcacgaggagacaactctaaggcgctagaatgctacatgaacgaaactggcgcttcggaagagatcgcgcgggaacatatcaggcatctggtccgggagacctggaagaagatgaacaaagaagtgtttgaggactacccattttccgggttcgggccttttcttagtgcctgtctaaacttggctcgagcttctcattgcttttacgagtatggagacggatatggccttcccgatcaccaaaccagggaccatcttgcgtcaactatattcgaatctgtgtcccttgattag

SEQ ID NO: 74 - DNA, 1620 bp, Artificial Sequence
  DNA having modified codons, which encodes linalool synthase gene derived from Backhousia citriodora (opt_BcLINS)
atgcgtcgctccgctaactggcagccctccgtgtgggattatgattatgttcaaagcctgaccgtggactataccgaagacaaatacaccaaacaagtgcagcggctgaaagaagaagttaaaggtttgtttgatcgcgaaatgaaacaagtggccaaattggaatttattgacgtggttcagcgcttggggctgggataccattttaaaactgaaattaaaattgccttgtccagtattcacaataacaccgaagatgctcaattgagcaatgacttatatgccgcttctttacggtttcgcttgttacgtcaatacggttgtaacgtgcaacaggatgtttttcagcggtttatgaacaaaaccgggacttttaaagaatccctgaacaaagacgttaaaggtattctggggttgtatgaagccagttttcatggaatggaaggcgaaaccgtgttggatgaagcctggaactttgcttccaaacacctgaaagatctgaacctggacgaagtgcccaccaatctggcctccaacgttagtcatgctttggatatgcccattcactggcgccccaatcgtttggaagcccgttggtttatggatatgtacgaaaaacaacaggacctgattcccagtctgttgcggctggctaaattggattttaacattgtgcaatccattcatcgcaaagaagttagtaatttagcccgttggtgggtggaactgggggctaacaaaatgacctttttccgtgatcggctggttgaaagctacttttggtcttgtattttggtgtttgaaccccagtacaccgactttcgggaattaaatactcgcattgcctgcatggctaccctgattgatgacgtgtatgatatttacggcactcccgaagaactggaactgctgaccgattttattctgcgctgggacattactgatattgacaaactgccccccaccattcgtaatggttttatggccttgtataataccactaacaaagtgggttaccgtaccatgactaaacgggggattaatcccattccctatttacggaaactgtggggagatgaatgtaaagccgacatgaaagaagtgcattggtttaataacgggattaaacccaccttaaaagaatacatggatgtggccgttgactccattggcggtctgattttgctgctgaatagttattttctgaccactgattacttgaccgaagaaggcttaaactatgtgtccaaaattcccagtgttatgcatagctctgcccaaatttttcggtttaatgatgacttgagcacctccagtcacgaattagcccgcggagataattctaaagctttggaatgctacatgaacgaaactggcgcctccgaagaaattgctcgggaacatattcgccacttagttcgtgaaacctggaagaaaatgaacaaagaagtgtttgaagattacccctttagcggctttggtccctttttgtctgcctgtttgaacttagcccgcgctagccattgcttttatgaatacggggatggatacggcttgcccgatcatcaaactcgtgaccacttagccagtaccatttttgaaagcgtgtctttagattaa

SEQ ID NO: 75 - DNA, 27 bp, Artificial Sequence
  Primer
tgtgaaattaaataccttgaatggggg

SEQ ID NO: 76 - DNA, 45 bp, Artificial Sequence
  Primer
gtatttaatttcacacaggagactgccatggattttccccagcag

SEQ ID NO: 77 - DNA, 28 bp, Artificial Sequence
  Primer
tgtgaaattaatctaaagacacgctttc

SEQ ID NO: 78 - DNA, 45 bp, Artificial Sequence
  Primer
tagattaatttcacacaggagactgccatggattttccccagcag

SEQ ID NO: 79 - DNA, 56 bp, Artificial Sequence
  Primer
aaggaattataaccaaatgtccaccgccgtgccctctatgcccactacccaaaaat

SEQ ID NO: 80 - DNA, 55 bp, Artificial Sequence
  Primer
ggcatggaggacatattagctactggaatcatacaacatggttttcatgtgttct

SEQ ID NO: 81 - DNA, 55 bp, Artificial Sequence
  Primer
tctagagtcgacgtcccctgttgacaattaatcatcggctcgtataatgtgtgga

SEQ ID NO: 82 - DNA, 55 bp, Artificial Sequence
  Primer
atccaatgtgaggttctatttgttgcgctggatgatgtaatcggccagggcttcc

SEQ ID NO: 83 - DNA, 45 bp, Artificial Sequence
  Primer
ttggaacattgtgttcagcccatggctgtctcccgccattgctaa

SEQ ID NO: 84 - DNA, 45 bp, Artificial Sequence
  Primer
ttgttcccggtacaacttagccaccaactccttgagaatgaccac

SEQ ID NO: 85 - DNA, 25 bp, Artificial Sequence
  Primer
ggaggattgggttaccctcagtgtg

SEQ ID NO: 86 - DNA, 25 bp, Artificial Sequence
  Primer
cgccatatcaatcccaacgctctgg

SEQ ID NO: 87 - protein, 299 aa, Escherichia coli
MDFPQQLEACVKQANQALSRFIAPLPFQNTPVVETMQYGALLGGKRLRPFLVYATGHMFGVSTNTLDAPAAAVECIHAYSLIHDDLPAMDDDDLRRGLPTCHVKFGEANAILAGDALQTLAFSILSDADMPEVSDRDRISMISELASASGIAGMCGGQALDLDAEGKHVPLDALERIHRHKTGALIRAAVRLGALSAGDKGRRALPVLDKYAESIGLAFQVQDDILDVVGDTATLGKRQGADQQLGKSTYPALLGLEQARKKARDLIDDARQSLKQLAEQSLDTSALEALADYIIQRNK

SEQ ID NO: 88 - protein, 299 aa, Artificial Sequence
  Mutant farnesyl diphosphate synthase derived from Escherichia coli whose 80th serine residue of the enzyme is substituted with a phenilalanine  (ispA* (S80F))
MDFPQQLEACVKQANQALSRFIAPLPFQNTPVVETMQYGALLGGKRLRPFLVYATGHMFGVSTNTLDAPAAAVECIHAYFLIHDDLPAMDDDDLRRGLPTCHVKFGEANAILAGDALQTLAFSILSDADMPEVSDRDRISMISELASASGIAGMCGGQALDLDAEGKHVPLDALERIHRHKTGALIRAAVRLGALSAGDKGRRALPVLDKYAESIGLAFQVQDDILDVVGDTATLGKRQGADQQLGKSTYPALLGLEQARKKARDLIDDARQSLKQLAEQSLDTSALEALADYIIQRNK

SEQ ID NO: 89 - DNA, 1575 bp, Arabidopsis thaliana
atggcaaatactgctaaaagatcgatcttgagaaacgtccatgcttcagtttctaacccttcgaagcagtttcataataagacatccttagaatatttacacgagttgaatatcaagaagatcaagaatatactaagtgcaaacgtagatgttccatccgagaacctggagatgatcgatgtcattcaaagtttaggcattgatctccattttcgacaagagatcgagcaaacccttcacatgatttacaaagaaggcctccaattcaacggtgatctccatgagatagcgcttcgctttcgattgctgagacaagagggtcactatgttcaagaaaacaagaagggtggatttaaagacgtagtaaaaaatgacgtcaagggtctaacagaattgtttgaagcttctgagctccgtgtagaaggtgaagaaacactcgacggtgcgagagaattcacatatagccgccttaatgaactttgctcaggtagagaaagtcatcaaaagcaagagataatgaagtctttggcgcaacctcgccacaaaaccgtaagaggattaacgtccaagaggttcacaagcatgatcaaaatcgcgggtcaagaagatccagaatggttacagtctctattacgagtggcggagatcgattccattaggctaaagtcattgactcaaggagaaatgtctcaaacatttaaatggtggacagaacttggtttagaaaaagatgtggagaaggcaagaagccagccgttaaaatggcatacgtggtccatgaaaattcttcaagatccgaccttaaccgaacaaaggcttgatcttaccaaaccaatatcgcttgtttatgttatagatgacattttcgatgtctatggggagctagaagaactaaccatcttcacacgagttgttgagagatgggatcataaggggcttaagacgctacccaaatacatgagggtttgttttgaagctctagatatgatcacaacggagattagcatgaagatctacaaatcacatggttggaacccgacatacgctcttcgacaatcgtgggcaagtttgtgtaaagcattcttggtagaagcaaagtggtttaattcgggttacttacccaccactgaagagtatatgaagaatggggttgtgagttcaggtgttcatttagtgatgcttcatgcctatatcttgttaggcgaagaactaacaaaagagaaagtcgaactaatagagagtaacccggggattgtatcatctgcagctacaattctcaggctctgggatgatctcggaagtgccaaggatgagaaccaagatggaactgatggatcatatgtagagtgttacctgaacgagtacaagggatcaactgttgatgaagcaagaacacatgttgcccagaagatatctagagcatggaaacgcttgaacagggagtgtctgaatccatgtccattctcaagatcattctcaaaagcttgtctcaacattgcaagaacagttcctttaatgtacagctatgatgatgatcaacgacttcccgacgaatatctcaagtctctaatgtaa

SEQ ID NO: 90 - DNA, 1644 bp, Arabidopsis thaliana
atgcgtcgttctgcgaactatcagccttctcgttgggaccatcaccatctcctctcggtcgaaaataaatttgcgaaagataaaagggtacgagagagagatttgttgaaggaaaaagtgagaaagatgctcaatgatgagcaaaagacttatcttgaccaattggagttcattgacgatctacaaaaactcggggtttcttatcattttgaagcggaaatcgacaacattttaacatcttcttataaaaaagatagaacaaacatccaggagagtgacctacatgccaccgcactcgagttccgacttttcaggcaacatggtttcaatgtttcagaagatgtattcgatgttttcatggaaaattgtgggaagtttgaccgtgatgatatatatggtttaatatctctttacgaagcatcatatctttcgacaaaattggataaaaacctgcaaatattcatcagaccttttgctacacaacaactcagagactttgttgatactcatagtaatgaagattttgggtcgtgtgacatggtggaaattgtggtccaagcgttggatatgccctactattggcaaatgagaaggctatccaccagatggtacatagatgtgtatggaaaaagacaaaattataagaaccttgtcgtcgttgaatttgccaagattgatttcaacatcgtacaagctattcatcaagaggaactcaaaaacgtttccagctggtggatggagacaggtttaggtaagcaactctactttgcaagagacagaatagtggagaattatttctggacgattggacaaatccaagagcctcaatacggatacgttcgacaaacaatgacgaaaataaatgcactccttactacaattgatgatatctacgatatctatggcactcttgaagaacttcagcttttcactgtcgcgtttgaaaactgggatataaatcgtcttgatgaactccccgagtacatgaggttgtgttttcttgttatatacaatgaagtcaatagcattgcatgtgagattctcagaactaaaaatatcaacgtgatcccattcctcaaaaaatcttggacagatgtatccaaagcgtatttagtagaagcaaagtggtacaaaagtggtcacaaaccaaatttggaagagtacatgcaaaatgctcggatttcaatctcgtccccaacgatatttgttcacttctactgcgtattctccgaccagctctctattcaggtcttggagactttgtcccaacaccaacaaaacgtcgtccgatgctcctcctcagtgttccgtctagccaacgaccttgtaacctcaccggatgaattggcgagaggagacgtctgcaaatccatccaatgttacatgagtgaaactggagcatcagaggataaggcgcgttcgcatgttcgacagatgatcaatgacttgtgggatgaaatgaattatgagaaaatggcacatagctcttcgatactccatcatgattttatggaaacagtgataaatttggcacgcatgtctcaatgcatgtatcaatatggcgatggccatggctctcccgaaaaagccaaaatcgttgatcgtgtcatgtccttactcttcaatccgattcctttagattga

SEQ ID NO: 91 - DNA, 1698 bp, Citrus unshiu
atgttgtttcaagtttcagcctctcctaataaagttatccgaataaatgccgagaaagaatctactcgtcgttcggcaaattttgatcctaccatttggggggattatttcctttcatatactggtgacttcaaggaaagtggtgatgctagcgtgaagcatcaagagctgaagaaagaaattagaacgatgctaagagctgatatcaacaagcctacgcagactaaactggatttgattgatgacattcagcgtttaggagtgtcttatcattttgaaagtgagattgatgaaatcttgcgaaaaatgcatgaggctaaccaagattgtgatcttggcgatgatgaaaatgttcaggagctctattatatctctcttcattttcgattacttagacaaaatggctataaaatttctgctgatgtctttaacagcttcaaggatagcaatgggaacttcaagtctttccttaaaagagatattcggggaatgttaagcctgtatgaagcggcacatctcagggtacatggagaaaatatactcaacgaagcacttactttcactgtcactcaccttgagtcatttacaagccaatccaacactcaacttgcggctcaagtcaatcgtgccctcaatcgacctattcgcaaaagcttaccaaggctagaggcaaaacactacatgccaatctatcagaaagacccttcacacaacaaagatctattaacctttgccatgttagatttcaacatacttcagaaacaacaccaagaagaactcagagatatcgtaaggtggtggaaaaattttgatgttcccaataagctacctttcataagagacagagtggtggagggctatttctggattttgggagtatattttgagccaaaatttttattggctagaaaaattctaaccaaagtgatatcaatggcttcaattattgatgacatttatgatgcttatggtacaatagaagaacttgagctttttgccacagcaattgagaggtgggatctcagtgccatagatctgcttcctgagtacatgaagttgtgctattgcgctctcctggatgcttacagcgaatttgagaaagatttggccagcaaaggaatattgtacggcctaccttttgctaaagaatcgatgaagattttggtgagaagttacatcatcgaagctagatggtgtgaccaacaatatgtaccgacaatggaggaatacatgcgcgttgcactactttcatgtggctacttactgttatcaacatcttcatttctgggaatggaagatattgtaacaaaagaagcctttgaatgggtatccggcaaccctaaaatcgttcaggcttcctcaataatttgcagactcatggatgacattgtctctcataagtttgagcaacagagaggacatgtggcctcagctgttgaatgctacatgaagcagcatggagtttctgaggaagaggcagttaaagtgtttcgggagaaagttgggaatgcgtggaaagatataaatgaggagctcatgagaccacctgttgttcctatgcctttgctcgaacgggttcttaatcttgctcgtttaatggatgtgctgtaccaaaataatgattcctatacaaatcctcacttgatgaaagatcatgtagccgcattgcttaaggatcctgttttctttgaagactag

SEQ ID NO: 92 - DNA, 1746 bp, Citrus unshiu
atggctttctcttccaaagatatttcgtctgattcatcccacattcactttattccaaaacacatatcaaaagttggcaaccgaaacctcaataacattaattctttgctgcctaataataaaaagggcagcattaatgataacataggtgtttctgcccggttgaaacgtttcacttatcccagtgaacactccagtaattttaatgacgacattcacattaagcatgcgaaaaaactggaggtaatcaagcacatacttatcaaactaggagatgacgattcttttgaaggattggccatgattgatgtcgttcaacgcctagggattgattactattttcaagatgagattgaactaattctacgaaggcagtatagcatatttttcactgatggtgatcgctataatgaccttcaagaggttgcccttcgctttcgactgttgagacaacaaggttactatgtgtctgcagatgtttttaacaggttcagaaacaaagaaggggagtttaaacagaatataagtgaagacatcaatggattgatgagcttatacgaggcctcacagctaagtattggaggagaagatgggcttgatgaagctggacactttagtgcgacacatcttgctaattatgatctagcgggagtagttgagcatctgttgctgtatccctatcgcaaaagcttgtccccggccaaaaactttttccatggcaattttcaaggcagtgaatatatttggatactggatttgcaagaactagcgaatatggatttcaaattggtccaatccttacaccaaaaggaaattgtgcaaatatccagttggtggagagagctcggtttggctaagaagttggaatttgcaagagagcaaccagttaaatggtatgtgtggtcaatggcatgtttcacggatccaaacttgtcgtggcaaaggatagagctcacaaaacccatctccttcgtctacattattgacgacattttttatgtttgtggagcactcgatgccctcacccttttcacagaacccattaatagatgggatcttggggacattgatcaattgccagagtacatgaagatatgtttcaaggctcttaacgatatcactaatgaaatcagcaaacaaggtgtacaaaggagcatgggtataaccctgtgcactcctttgcgaaagggcgtgggggaagttttgtgcaacgcgttcctaatagaggcaaaatggtttgcttccgggcacttgcctaaggctgaagagtacttggaaaatgggattgttagttcaggggtacacttggtacttgtgcacattttctttctcctgggtcatggcatcaccaatgaaacagtgcaactcattgacagcaacccacccattgtatcatccgtcgcaacaattcttcgaatttgggatgacttgggaagtgctaaggatgaaaatcaaggcggcaaagatggatcatatatatattactacatgatggaacaccgagacttaacggctgaagatgcacacaagcatgccatggataagatttcagatgcatggaagcgcctaaacaaggaatgcctctccccaaatccattttcagcatctttcacaagggcttcttttaactgtgccagaatggttcctttgatgtacagctatgatgacagccaacggcttccgagcctcgaggagtatattaagtcctccctttttgataatttgcctactcaaggagtgtactag

SEQ ID NO: 93 - DNA, 1767 bp, Citrus unshiu
atggctttctcttccagttctagagctaagttgtctgctacctcccacatttcaaaggctccagataagatttcaaaaactagcaggcctagcctcattgaatttactccttcgcctactatctatcaaaaagggtgcattactagtgacaatacagtcgcttctcctccccttaaacacttcacccacacaactagacaccccagcttcttcgatcatgatattcaagtcgaacattctcggaaattgaaggaattcaagcatatatttagcctagtcgggggaaattcttttgaaggattagtcatgattgatgctgttcaacggctacgcattgagtaccttttcaaagatgagattgaagaaattttacaaaggcaatatatcatatcttccacttgtggtggtcacctccatgatcttcaagaggttgcccttcgctttcggttgctgagacaagaaggttactacgtgcctgcggatatgtttaacaactttaggatcaaggaagggagattcagccggatcaacgtaagtgaagacatagggacattgatggaagtatatgaagcttcgcagctaagtatagcaggcgaagaagggcttgacgaagccggacactttagtgcgaagatgctcaatgagtgcatgacacatcttgatcactatcatgctctagctatcgggaatactttgaggcatccataccacaaaagcttgcccagatttatggccaaagacgttttccttagcaatttccaaggtgaacgcagattgcatgttttaaaagaaatagcgaaaaaagatttcaacatggtacaggccttacaccaaaaagagattgttcaagtaaccaaatggtggaaagacctcggtttgactaagaagttgccgtttgcaagagaccaaccacttaaatggtacatttggtctatggcttgcctcacagatccaagcttgtcagagcaaagagttgagctcacaaaacccatatccctcatctacattattgacgacatatttgatgtttatgggacgcttgatgaacttattctcttcacagaaactattactagatgggatcttgccgctatgggtcaattgcctgagtacatgaagatatgtttcaaagctcttgacgatattactaacgaaatcagctgcaaggtctataagaagcatgggtataacccagtacagtccctccgaaatgcgtggacaagtttgtgcaaagcatttctagtggaagcgaaatggtttgcttctggacacatgcctgaggctgaagaatacttgaggaatgggattgagagttcaggagtacatgtggcactggcgcactttttttttctcctaggtcatggtataactaaggaaacggtggagcttattgacggtaacccggccataatatcatcaaccgcaacaattcttcggctctgggatgacttgggaagtgcaaaggatgagaatcaagaaggtaaggatggatcttacatccattactacatgaaggaacaccgatattctgccgccgaagaggcacaaaaaagtgctatcaataaaatttcagacgcatggaagcggctcaacaaagaatgcctctgcccaaatccattctcagcatctttcacgagggcttctctcaatcttgcaagaatggtccccttgatgtacagttacgatgacaaccaacgcctaccaagcctcgaacattacattaagtccctactctttgaaagcgtacctactgaaggagtttattaa

SEQ ID NO: 94 - DNA, 1704 bp, Malus domestica
atggaattttctatttcccagtcctcctttgcgacctcgtcttctactccagctgctccggaacaccttagttctcaaaaatggagcatccccgaagatcacagtttgctttctactcccttaaaaccgcttaactccaaaacgaagtatacttcatctaaggatggcataatttgtttccagaatgaacaaaaactggacgacttaaggcatgcattgataaaagtgggaggagaagcagttgaaagtttggacatgatcgatgcggttcaacggctaggtctagactaccactttgaagaagaaattgaccaaattctccaaaagcaacatataatatctagtactactgctcatggtgctcaccatcccaccgacctacatgaagtcgctctccgctttcgactactcaggcagcatggttacttcgtctctgatgatgtgtttaacaacttcaagaacagagaaggaaatttcaatcaaatgttaagggaagacatcaaggggttgatgagtttgtatgaagcttcacagctaagtatagagggtgaagttgtacttgaagaagctggaaagtttagtggccatttcctaaattcatcactgtcacatctcgatcatcaccaggccagagttgttggaaacacattgagaaatcctcatcacaaaagcttggccccattcatggccaagaacttttttgtctctagcttccaaggaacaaataatagatggctaaatatattacaaactgtagcaaaaacagatttaaatatggtccagtcccttcaccagaaagaagttgctcaagtttccaaatggtggaaagagctgggattgtgtaaggagttgaagtttgcaagagaccaacctattaaatggtacatttggtccatggcttgcctaacaaatccaaacttgtcagatgagaggattgagctcacaaaacctatctcatttatctatttgattgatgacatttttgacgtttacgggacgcttgatgaactcactcttttcacggaggttgtcaatagatgggaaattggttctatagagcacttaccggactacatgaagatatgcttcaaggctctttacgatatgacgaatgaaatcagctgtaaggtctatcaaaagcacggatggaacccattgcattcgctaaagaagacgtgggctagtctgtgcaatgcatttttagtggaagcaaaatggttcaaatctgggcacttgcctatggctgaagagtacttgaagaatggaattatttcttctggggtgaatgtggtgatggtccacattttctttctgttgggtgaaggtataaccaatcaaagtgtggagttcttgaatggcactccagccattatatcttcaacggcagcaattcttcggctttgggacgacttgggaagtgccaaggatgagaatcaagatggggacgacgggtcatatgtaaagttgtatttaaatgaacatcaaggcaagaccatggaggaagcacaagaacatgttacaaatatgatttcagaagaatggaagaagctgaacaaagaattggtgtctcctaatccacttcccgcggcattcacaaaggcttccctaaatctcgcaagaatggtgccattgatgtatagctacgacgacaaccagtgccttccatctcttgacgagtacatgaaatcgatgcttcatgcatga

SEQ ID NO: 95 - DNA, 1824 bp, Perilla frutescens var. crispa
atgtatagcttgagaatatatgtagcgatcatgaaaaagccatcagctaaacatgttgacaacgtcgacaagaaagcttcaaagccgtcgtggcgtgtctcactctcttcgagtgcgggtctccgagcttcttcctccttacaactcgatgtaaaaaagcccgctgatgatgaaattctgacggcccgacgctctggcaactaccagccttccctttgggatttcaactaccttcaatctctcaacactactcagtataaggaagtgaggcacttgaaaagggaagcagagctgattgagcaagtgaagatgctgctggaagaagaaatggaggcagttcaacaattggagttggttgatgacttgaaaaatctgggattgtcttatttttttgaagaccaaattaagcagatcttaacgtttatatataatgagcataaatgtttccacagtaatagtattattgaagcggaggaaattagggatttgtatttcacagctcttggattcagactcctcagacaacatggtttccaagtctctcaagaggtatttgattgtttcaagaacgaggagggtagtgatttcaaagcaaggcttggtgacgatacaaaaggattgctgcaactctacgaagcctctttcctattgagagaaggtgaagatacactggagctagcaaggcaatatgccaccaaatttctccagaaaaaagttgatcatgaattaattgacgacaataatctattatcatggattctccattctttggagatcccgcttcactggaggattcagaggctggaggcaagatggttcttagatcgttacgcgacgagacgagacatgaatcaaatcattcttgagctcgccaaactcgacttcaatattattcaagcaacacaacaggaagaactcaaagatctctcaaggtggtggaagagtacatgtctggctgagaaacttccattcgtgagggataggcttgtggaaagctacttttgggccattgctctctttgaacctcatcaatatggatatcacagaaaagttgctgccaagattattacactaataacatctttagatgatgtttacgatatctatggtacattagacgaactacaactatttacagacgcgattcaaagatgggatactgaatcaataagccgccttccatattatatgcaattattttatatggtactctacaactttgtttcggagctggcttacgatggtctcaaggagaagggtttcatcaccatcccatatttacagagatcgtgggcagatttggttgaagcatatttaaaagaggcaaagtggttctacaatggatatgtaccaagcatggaagaatatctcaacaacgcctacatttcaataggggctactcccgtaatttctcaagttttcttcacattagcaacctccattgacaaaccagtgatcgacagcttgtacgaataccaccgcatacttcgcctctctggaatgcttgtaaggcttcctgatgatttaggaacatcaccgtttgagatgaagagaggcgacgtgccgaaagcaatccagttgtacatgaaggaaagaaatgctaccgagatagaggctcaagaacacgtgaggtttctgattcgtgaggcgtggaaggagatgaacacggtaacgacggcggccgattgtccgtttacggatgatttggttgcagcgacacgtaatcttggtagggcggcacagtttatgtatctcgacggagatggtaaccactctcaattacatcagcggattgcgtgcctactgttcgagccatatgcatga

SEQ ID NO: 96 - DNA, 1734 bp, Vitis vinifera
atgggattctctcctgccttttacgcttgctccattcctccagttggtcctaacaaattcacagagctaggccagtccaaattcaacaatgttgtgcttgtgcctactgctcagaaatggagcattgcccacgaccacaccttggtttataagcccttaagaaagcataatcatcaatctcaacatctcagctttactgatgaattttacatcaagcatgcacaaagattggatgaaattagaaacgtattcagtgaagttggagaggatacgctggaaggtttgatgatgattgatgccatacaaaggttgggcattgactaccacttcaaagaggaaattgaagcagttctacagagacagtatatgaaagccagcactcacggtgagagcattcaggatctctacgaggttgctcttcgttttcggctattgagacaagaaggttaccatgtgcctgcagatgtgtttaacaacttcaagaacaaggaggggaagtttaaacaaaatctcagcaaagacatcaagggattgttggctttatatgaagcttcacaactgagtatagaaggagaagatatcctcgaggaagcccaaagattcagcagcacgctccttaacgcagggttggaacatcttaatcaccacgaagctacagttgttgggcatacactggagcatccccatcataagagcttgccaaggttcatggccaaaagcttccttaaggacttccagggaccaaatggatggctgactgtcttgcaagaacttgcaaaagcggatttcaatatggttcaatccatacatcagcaggaattacttcaaatttcgaaatggtggcaagaccgaggtttggctgaggagttgaaatttgcaagagaccaaccactgaaatggcacatgtggcccatggcagtactccccgatccaagcttgtcagagcaaagggttgagctcacaaaacccatctctatgatctatataatcgatgacatttttgatgttcatggaacgcttgatgagctcactctctttacagaagctgtcaatagatgggatatagctgctttcgagacgctaccaaactacatgaagatatgcttcaagactctagatgaaatcacaaatgaaatcagcaacaaggtctacaaagagcacgggtggaacccagtagactcgctacggaagacgtgggtgagtttatgcaatgcgtttctagtagaagccaaatggtttgcctctgggcatgtgccaaaggcccacgagtacttgaaaaacggggtcatcagttcaggggtacatgtggtgcttgttcacttgttctttctcttgggccatggcataaccaggggaaatgtggatcttgtggatgacttccccagcatcatatcttccacagctgccattcttcgtctttgggacgacctgggaagcgccaaggatgagaatcaagatggccacgacgggtcatacatcgagtgctacattaaggaacaccaaggctcttccatggaaaatgcacggcaaaatgtgacctatatgatttcagacttatggaagcgcctcaacaaggagtgcctctctcagcatccattttcaacttcttttacaaagggttcccttaacattgcaaggatggttcctttgatgtacagttatgatgacaatcagagtcttccacaccttgaggaacatatgaagtccctcctctttgaagcatttcccctgtag

SEQ ID NO: 97 - DNA, 1809 bp, Vitis vinifera
atggaactaaccctcacatccctctcacccttggcctatggtgccctcaattgtcgtaaaaattttgccatggcatccccaagaatgagaatcaagcaagggagatcagaattgcccaacctcacaatcacttcgaagattgatgagttacaagtgaccgaaaggcgatcggctaattaccatcctagcatttgggaccccaaatttattgagtccttaagcactccctatacgaatgagggctattccaaccaattagaggacttgaaggaagaagctaaaagggtaattaaggacgctagagacacttcctcccgattagagttcattgattcgatgcaacggttgggagtggcttaccatttggaggaggagatcaaagaggctattgatcttgttcatttggatgataccactaccgatgatctttccacaactgcactccgatttagacttctacgacaacacggctatccagttagctcagaggtgtttgatcaattcagaagtaaagatgggagattcatggatggcatcagccaggatattgctgggcctttgagtttgtatgaagcttcccatcttggagtcgagggagaagatgacttggaagaagccaggaggttcagtactatacatttgaagtcactggttgggaatttggagagtgatttagctgaccaagtgcagcagtccctggaagttcccttacactggagaatgccaaggctagaagcccgaaacttcatcgatatctaccaaaggcgcaatacgaagaactctgctctccttgagctagccaagctggactacaatctagtgcaatcatcatatcagacggagttgaaggagctaacaaggtggtggacggacttgggatttaaggagaagctaagtttttctcgggatcgattgatggagaactatttgtggtcaatggggatcgctcctgagccccacttctccaaaagcaggataggactcaccaaattcatatgcatattaacagccatagatgacatgtatgacatatatggatcaccggatgagcttcgacgttttacagatgctgtgaatcgatgggatactgaggcactggtggaccttccagattacatgaagatatgttacttggccatgttcaactttgctaatgaaatggcctacgatgcattaagagatcacgacctatatattttaccctatcttaaaagtcagtggctaaatctctgtacatcctactcaatggaagctcaatggttttacaatgggtataagccaagcatcgatgaatacttaagcaatgcctggacttccgtagggggtcctgcagccatggtccatgcctattttctaatgggttgtgccaccaagggaaacttgaacaattgtttagacaatgcctctaatctactttattggtcatctcttattactcgacttagcgatgatttgggaacttctttagccgagattgcgagaggcgacgtggcaaaatctatccaatgttacatgattgaaaaatgtatatccgaagaacaagctcgagatcaagtagagaagcttatacgttactcatggaaaaagttgaatgaagcaagtactgatagctctctcccaaagtccttaataaattcatcattgaacatggcgcgatcagctcaatgtatttttcaatttggagatggaatcggtacatcagttggggtgaccaaagatcgattgacatcattcattatcaagccaatattgatagaaccaagcattaaaccctatcttgatggcatgaagatgagcaacagaagatga

SEQ ID NO: 98 - DNA, 1695 bp, Lavandula angustifolia
atgtcgatcaatatcaacatgcctgcagccgccgtcctccgcccttttcgctgctcacaactacatgtcgatgaaacccgacgctccggaaactaccgcccctcggcttgggattccaactacatccaatctctcaattctcagtataaggaaaagaagtgcttgacaaggctagaagggctgattgagcaagtgaaggaactgaaggggacaaaaatggaggctgttcaacaattggagttgattgatgactcgcagaatctgggattatcatattattttcaagataaaattaaacatatcttgaatttgatatataatgatcacaaatatttttacgatagtgaagctgaaggaatggatttgtattttacagctcttggatttagactctttagacaacatggttttaaagtctcccaagaagtatttgatcgtttcaagaacgagaatggtacgtatttcaagcacgacgatacaaagggattgttgcagctctacgaagcatcattcctagtgcgagaaggcgaagagacactcgaacaagcacgagaatttgccaccaaatccctacaaagaaaacttgatgaggatggtgatggaattgacgccaatatcgaatcatggatccgccactctctggagatcccacttcattggagggctcagaggctagaggcgagatggttcctagatgcttatgcgagaaggcccgacatgaaccccgttatcttcgagcttgctaaactcaacttcaatattgtccaagcaacacaacaagaagaattgaaagctctctcgaggtggtggagtagtttaggcctagctgaaaaactcccatttgtgagggataggcttgtggaaagctacttttgggctattccactctttgagcctcatcaatatggatatcaaagaaaagtggccaccaagatcataaccctaatcacatctttagacgatgtttacgatatctatggcacgttagatgaattgcaactatttacgaacttatttgaaagatgggataatgcatcaatcggccgacttcctgaatacttgcaattgttctatttcgcaatccacaactttgtttccgaggtggcttacgacattctcaaagaaaagggtttcactagtattgtatatttacagagatcgtgggtggatttgctaaaaggatacctaaaagaggcaaagtggtacaatagtggatacacgccaagcctcgaggaatatttcgacaacgcattcatgacaataggggcccctccggtactatcgcaagcttatttcacattaggaagctcgatggagaaaccgatcatcgagagcatgtacgaatatgacaacatacttcgcgtttcgggaatgctcgtgaggcttcccgatgacctaggaacatcatcgttcgagatggagagaggcgacgtgccgaaatcggtccagctatacatgaaggaaacaaatgctacggaggaggaggcggtggagcacgtgaggtttttgaatcgggaggcgtggaagaagatgaacacggcggaggcggccggtgattctccgttagtgagtgacgtggtggcggtggcggcgaatcttggaagggcggcgcagtttatgtatttcgacggagatggtaaccagtctagtttgcagcagtggattgtgagcatgctgttcgagccgtacgcatga

SEQ ID NO: 99 - DNA, 1821 bp, Mentha citrata
atgtgtactattattagcgtaaatcatcatcatgtggcgatccttagcaagcctaaagtaaaacttttccacaccaaaaacaagagatcagcttcaattaatctcccatggagtctctctccttcttcatccgccgcctctcgccccatcagttgttctatctcctcaaaactatataccatcagttcggctcaggaggaaacccgacgttccggaaactaccacccttcagtttgggattttgatttcattcaatctctcgacactgatcactataaggaggagaagcagttagagagggaggaagagctgatcatggaggtgaagaagttgttgggggcaaaaatggaggcaactaagcagttggagttgattgatgacttgcagaatttgggattgtcttattttttccgagacgagattaagaatatcttgaattctatatataaaattttccaaaataataatagtactaaagtaggggatttgcatttcacgtctcttggattcaggctcctccggcagcatggtttcaacgtttcacaaggagtatttgattgcttcaagaacgagcatggtagcgatttcgagaaaaccctaattggggaagatacgaaaggagtgctgcaactttacgaagcatcattccttttgagagaaggtgaagatacattggaggtagctagaaaattctccaccgaatttctcgaggaaaaactcaaagccggaatcgatggtgataatctatcatcatcgattggccattctttggagatccctcttcactggaggattcaaagactagaggaaagatggttcttagatgcttactcaaggaggaaagacatgaaccctatcattttcgagctcgccaaactcgacttcaatattattcaagcaacgcagcaagaagaactcaaagatctctcaaggtggtggaatgattcaagcctacctcaaaaactcccatttgtgagggataggctggtggaaagctactattgggcccttgggttgtttgaggctcacaaatttggatatgaaagaaaaactgctgcaaagattattaccctaattacagctcttgatgatgtttatgatatttatggcacactcgacgagctccaactatttacacacgtcattcgaagatgggatactgaatcagccacccaacttccttattacttgcaattattctatttcgtactatacaactttgtttccgaggtggcgtaccacattctaaaggaagagggtttcatcagcatcccatttctacacagagcgtgggtggatttggttgaaggatatttacaagaggcaaagtggtactacactaaatatacaccaaccatggaagaatatttgaactatgccagcatcacaataggggctcctgcagtaatatcccaaatttattttatgctagccaaatcgaaagagaaaccggtgatcgagagtttttacgaatacgacgaaataattcgcctttcgggaatgctcgtgaggcttcccgatgacctaggaacactaccgtttgagatgaagagaggcgacgtggcgaaatcaatccagatttacatgaaggaacagaatgcaacacgggaagaagcagaagaacacgtgaggtttatgattagggaggcgtggaaggagatgaacacaactatggcggcgaattctgatttgagaggtgatgtggttatggctgcagctaatcttggaagggatgcacagtttatgtatctcgacggagacggtaaccactctcagttacaacaccggattgcgaacttgctgttcaagccatatgtctga

SEQ ID NO: 100 - DNA, 1608 bp, Ocimum basilicum
atggcatccgcagtgcctctaagttcaactcctctcatcaacggggataactctccgcttaaaaacacacatcaacacgtggaggagaggagcagcaagaggagagaatatctgctggaggaaacggcgcgaaaactgcagagaaacgacaccgaatcggtggagaaactcaagctcatcgacaacatccaacggctgggaatcggctactattttgaggatgccatcgacgccgtactccgctcgcctttctccgccgaagaagaagaagacctcttcaccgctgctctgcgcttccgcttgctccgccacaatggcatccaagtcacccctgaaatattcctaaaattcaaggacgagagaggagaattcgacgaatcggacacgctagggttactgagcttgtacgaagcgtcaaatttgggggttacaggagaagagatactggaggaggctatggagttcgcggagcctcgcctgagacgatcactgtcagagctggcggcgccgcttcgtagtgaggtggcgcaagccctagatgtgccgaggcatctgagaatggcgaggttggaagccagacgattcatcgagcagtatggtaaacagagcgatcatgatggagaccttttggagctagcaattttggattataatcaagttcaggctcaacaccaatccgaactcactgaaattaccaggtggtggaagcaactgggtttggtggaaaagttgggtttcggtagagacagagcgttggagtgctttatgtggaccatggggatcctacctcaccctaaatactcttcttctagaatagaatcagccaaggcagctgctcttctgtacgtcatcgatgatattttcgatacctatggcaaaatggacgaactcatcctcttcaccgacgcaattcgaagatgggatttggaagcaatggagggtctacccgagtacatgaaaatatgctacatggcgttgtacaacaccaccaatgaaatatgctacagagtgctcaaggatactggacggatcgccctcccatacctcaaatctgtgtggatagagactattgaagcttatatggtggaggtgaagtggttcagtggtggaagtgccccaaagttggaagaatacattgagaatggggcatcaactgtaggggcatacatggttcttgtccacctattctttctcattggagaaggtctcacccaccaaaatgtcctatttttcaaacaaaaaccctatcacaagcctttctccgccgccggccggatttttcgcctttgggacgatcttggaacttctcaggaggaggaagaacgaggagatatggcgtcaagtatacggttatttatgaaagagtacaagttgtcgacggtagaggaggctagaagttgcgttttggaagagatatcccgtttatggaaggatcttaatgaagggctcatcagtataaaggacgccttgccattaaccatagtcaaagtcgcacttaacattgcacgaacttctcaagttgtatacaagcacgaacaacatacatatatgttgagtgttgataattacgtggaagccctcttcttcactcctcttctttcttcttag

SEQ ID NO: 101 - DNA, 2550 bp, Clarkia breweri
atgagagaatcattgtcttcttcatcatctaatactcagaatttgtttctctcaacttcaccttatgacactgcttggctcgcccttatccctcatcctcatcatcaccatcaccatggccgacccatgtttgaaaaatgtctgcaatggattctccataaccagacaccacaaggtttctgggcagcagctggtgacaatatttccgacaccgacgatgacgtcaccctggattgtcttctatcaaccttggcttgcttagttgcactcaaaaggtggcagcttgctcccgacatgattcataaaggattggaatttgtaaatagaaacacagagagacttgtaatgaagcagaagccgagcgacgttcctcgttggttcaccatcatgttcccggcgatgctcgagcttgccggagcttccagtctccgagtcgatttcagcgagaatcttaacagaatcttggtggaactatctcaaaatagggatgatattctcacaagggaggaagttgatgagaagaagcaatactcaccattgctactatttctagaagcattgcctgcacaatcctatgacaatgatgttctaaagcaaattatagacaagaacttgagcaatgatggttctttattgcaatcgccttctgctacagcaagagcatacatgataacaggaaataccagatgcttatcgtatctacactctttaacaaatagctgctctaatggaggagtaccatcattctatcctgttgacgacgacctccatgatcttgtcatggtgaatcaactgacaaggtcgggtttgactgaacatctcatcccggagattgaccaccttctactcaaagttcaaaagaactacaaatacaaaaaagcatcaccaaaatcattgtatagcattgctgcggaactatacagggattcattagcattttggttgcttcgagtcaataatcactgggtatcaccatcaattttttgttggtttttagatgacgacgaaatccgtgatcacatcgaaacaaactacgaggaatttgctgccgtgcttcttaatgtgtatcgagctaccgatcttatgttctccggcgaagtccaacttgtcgaagcaagatctttcgctaccaagaatcttgagaaaatattagcaacaggaaacatacataaaactaatgcagatatctcatctagtttgcataagatgatcgaacacgaactaagagttccttggaccgcaagaatggaccatgttgaaaatcgaatttggatcgaagaaatagcttccagtgctttatggtttggaaaatcatcctaccttaggttatcttgctttcacaagatgagtttacagcaactcgcggtgaaaaattatacgcttcgacaattggtttaccgagacgagcttgcggaagttgagaggtggtctaaagaaagagggctatgtgacatgggattttgtagagagaaaaccgggtattgttactacgcatttgcggcaagtacttgtctgccgtggagttccgacgtgaggctggtcctgaccaaggcggcagttgtcattacagtggccgatgatttctttgatgtcgaaggatctatggttgatctcgaaaaattaacggatgcagttcggaggtgggatgcggaagggttaggcagccacagcaagacaatatttgaagccctggatgatcttgtaaatgaagttagactcaagtgtttccaacaaaatggacaagacatcaaaaacaatctccaacaattatggtatgaaacattccattcatggcttatggaagctaagtggggaaaggggttaacaagtaaaccatctgtagatgtgtatcttggaaatgcaatgacatccatagcagctcacaccatggtccttacagcatcctgtcttctaggtcccggtttcccggttcaccaactatggtcgcaaaggcgccaccaggacattacatccttgctcatggtcttgactcgcttgctaaatgacattcaatcctacttgaaagaagaagacgaaggaaaaataaactatgtatggatgtacatgatcgagaacaatcaagcgtcgatagatgactcggttcgacacgtccagacgataatcaatgtaaaaaagcaagaattcatccaacgtgttctatcggatcaacattgcaatctcccaaagtcattcaagcagctccatttctcctgcctcaaagtattcaacatgttcttcaactcctccaacattttcgacactgataccgaccttcttcttgacattcacgaagcttttgtttctccaccacaagttcccaaattcaaaccccacatcaagccacctcatcagcttccagcaacacttcagccacctcatcagccccaacaaataatggtcaataagaagaaggtggaaatggtttacaaaagctatcatcatccattcaaggttttcaccttgcagaagaaacaaagttcgggacatggtacaatgaatccaagggctagtatcttagcaggacccaacatcaaactatgtttcagttaa

SEQ ID NO: 102 - DNA, 1575 bp, Artificial Sequence
  DNA having modified codons, which encodes linalool synthase gene derived from Arabitopsis thaliana (At1LINS)
atggcgaacacggcgaagcgtagtatcctgcgtaatgtccatgcgagcgttagcaacccgagtaagcagtttcataataagacgagtctggaatacctgcatgaactgaacattaaaaagatcaagaacattctgagcgccaatgttgacgtgccgagcgaaaatctggaaatgatcgatgtgattcagagcctgggcattgacctgcattttcgccaggaaattgaacagaccctgcacatgatctacaaagaaggcctgcagtttaatggcgatctgcatgaaattgccctgcgttttcgtctgctgcgtcaggaaggccactacgtccaggaaaataaaaagggcggctttaaagatgttgtgaagaatgacgtgaaaggcctgacggaactgtttgaagcgagcgaactgcgcgtcgaaggcgaagaaacgctggacggcgcccgcgaatttacctacagccgcctgaatgaactgtgtagcggccgcgaaagccatcagaagcaggaaattatgaaaagcctggcccagccccgtcacaaaacggttcgcggcctgacgagcaagcgctttaccagcatgattaaaatcgcgggccaggaagatcccgaatggctgcagagcctgctgcgcgtggccgaaatcgacagcattcgcctgaagagcctgacccagggcgaaatgagccagacgtttaaatggtggaccgaactgggcctggaaaaggatgttgaaaaagcgcgcagccagccgctgaagtggcatacgtggagcatgaaaattctgcaggatccgaccctgacggaacagcgcctggacctgaccaagcccatcagcctggtctacgttatcgatgacatttttgatgtctacggcgaactggaagaactgaccatctttacgcgcgtcgttgaacgctgggaccataaaggcctgaagaccctgcccaaatacatgcgcgtttgttttgaagcgctggatatgatcaccacggaaattagcatgaaaatctacaagagccacggctggaatcccacctacgccctgcgccagagctgggccagcctgtgcaaggcgtttctggtggaagccaaatggtttaatagcggctacctgcccaccacggaagaatacatgaagaatggcgtggtcagcagcggcgtgcatctggtcatgctgcacgcgtacattctgctgggcgaagaactgacgaaagaaaaggtcgaactgattgaaagcaatccgggcatcgttagcagcgcggccaccattctgcgtctgtgggatgacctgggtagcgccaaggacgaaaatcaggatggcacggacggcagctacgttgaatgttacctgaatgaatacaaaggcagcacggttgatgaagcgcgcacccacgtggcccagaagattagccgcgcgtggaaacgcctgaatcgcgaatgtctgaatccgtgcccctttagccgcagctttagcaaagcgtgcctgaatatcgcccgcacggtgcccctgatgtatagttatgatgatgaccagcgtctgcccgatgagtatctgaaaagcctgatgtaa

SEQ ID NO: 103 - protein, 524 aa, Arabidopsis thaliana
MANTAKRSILRNVHASVSNPSKQFHNKTSLEYLHELNIKKIKNILSANVDVPSENLEMIDVIQSLGIDLHFRQEIEQTLHMIYKEGLQFNGDLHEIALRFRLLRQEGHYVQENKKGGFKDVVKNDVKGLTELFEASELRVEGEETLDGAREFTYSRLNELCSGRESHQKQEIMKSLAQPRHKTVRGLTSKRFTSMIKIAGQEDPEWLQSLLRVAEIDSIRLKSLTQGEMSQTFKWWTELGLEKDVEKARSQPLKWHTWSMKILQDPTLTEQRLDLTKPISLVYVIDDIFDVYGELEELTIFTRVVERWDHKGLKTLPKYMRVCFEALDMITTEISMKIYKSHGWNPTYALRQSWASLCKAFLVEAKWFNSGYLPTTEEYMKNGVVSSGVHLVMLHAYILLGEELTKEKVELIESNPGIVSSAATILRLWDDLGSAKDENQDGTDGSYVECYLNEYKGSTVDEARTHVAQKISRAWKRLNRECLNPCPFSRSFSKACLNIARTVPLMYSYDDDQRLPDEYLKSLM

SEQ ID NO: 104 - DNA, 1644 bp, Artificial Sequence
  DNA having modified codons, which encodes linalool synthase gene derived from Arabitopsis thaliana (At2LINS)
atgcgtcgtagtgcgaattaccagccgagtcgttgggaccatcatcacctgctgagtgtggagaataagtttgcgaaggacaagcgtgtccgcgaacgcgacctgctgaaagaaaaggttcgcaaaatgctgaatgacgaacagaagacctacctggatcagctggaatttattgatgacctgcagaaactgggcgtcagctaccattttgaagccgaaattgataatatcctgaccagcagctacaaaaaggaccgcacgaatatccaggaaagcgatctgcatgccacggcgctggaatttcgcctgtttcgccagcacggctttaatgttagcgaagatgtgtttgacgtctttatggaaaattgtggcaagtttgaccgcgatgacatctacggcctgattagcctgtacgaagccagctacctgagcaccaaactggataagaatctgcagatttttattcgtccctttgccacccagcagctgcgtgattttgttgacacgcatagcaatgaagattttggcagctgcgacatggtggaaattgttgtgcaggccctggacatgccctactactggcagatgcgccgcctgagcacccgttggtacatcgatgtgtacggcaaacgccagaattacaagaatctggtcgttgtggaatttgccaaaatcgactttaatattgtgcaggcgatccaccaggaagaactgaaaaatgtcagcagttggtggatggaaaccggcctgggcaagcagctgtactttgcgcgcgatcgcattgtcgaaaattacttttggacgattggccagatccaggaaccgcagtacggctacgttcgccagaccatgacgaagatcaatgccctgctgaccacgattgatgacatctacgatatttacggcaccctggaagaactgcagctgtttacggttgcgtttgaaaattgggatattaatcgcctggacgaactgccggaatacatgcgcctgtgttttctggttatctacaatgaagtgaatagcattgcctgcgaaatcctgcgcaccaagaacatcaacgtgatcccctttctgaaaaagagctggacggacgtgagcaaagcctacctggtcgaagcgaaatggtacaagagcggccataagccgaatctggaagaatacatgcagaatgcgcgcattagcatcagcagccccaccatctttgtccatttttactgtgtttttagcgatcagctgagcatccaggtgctggaaacgctgagccagcaccagcagaatgtcgttcgctgcagcagcagcgtttttcgcctggccaatgatctggtgaccagccccgatgaactggcccgcggcgatgtgtgtaaaagcattcagtgctacatgagcgaaacgggtgccagcgaagataaggcccgcagccatgtccgccagatgatcaatgatctgtgggacgaaatgaattacgaaaaaatggcccacagcagcagcattctgcatcacgactttatggaaaccgttatcaatctggcgcgcatgagccagtgtatgtaccagtacggtgatggtcatggcagccccgaaaaagccaaaatcgtggaccgtgtgatgagcctgctgtttaaccctatcccgctggactaa

SEQ ID NO: 105 - protein, 547 aa, Arabidopsis thaliana
MRRSANYQPSRWDHHHLLSVENKFAKDKRVRERDLLKEKVRKMLNDEQKTYLDQLEFIDDLQKLGVSYHFEAEIDNILTSSYKKDRTNIQESDLHATALEFRLFRQHGFNVSEDVFDVFMENCGKFDRDDIYGLISLYEASYLSTKLDKNLQIFIRPFATQQLRDFVDTHSNEDFGSCDMVEIVVQALDMPYYWQMRRLSTRWYIDVYGKRQNYKNLVVVEFAKIDFNIVQAIHQEELKNVSSWWMETGLGKQLYFARDRIVENYFWTIGQIQEPQYGYVRQTMTKINALLTTIDDIYDIYGTLEELQLFTVAFENWDINRLDELPEYMRLCFLVIYNEVNSIACEILRTKNINVIPFLKKSWTDVSKAYLVEAKWYKSGHKPNLEEYMQNARISISSPTIFVHFYCVFSDQLSIQVLETLSQHQQNVVRCSSSVFRLANDLVTSPDELARGDVCKSIQCYMSETGASEDKARSHVRQMINDLWDEMNYEKMAHSSSILHHDFMETVINLARMSQCMYQYGDGHGSPEKAKIVDRVMSLLFNPIPLD

SEQ ID NO: 106 - DNA, 1698 bp, Artificial Sequence
  DNA having modified codons, which encodes linalool synthase gene derived from Citrus unshiu (Cu1LINS)
atgctgtttcaggtgagcgccagtcccaataaggtgatccgtattaacgccgagaaggagagtacccgtcgtagtgccaactttgacccgacgatttggggcgattactttctgagctacaccggcgattttaaagaaagcggcgacgccagcgtcaagcatcaggaactgaaaaaggaaattcgcacgatgctgcgcgcggatatcaataaacccacccagacgaagctggacctgattgatgacatccagcgcctgggcgtgagctaccattttgaaagcgaaattgacgaaatcctgcgcaaaatgcacgaagccaatcaggattgtgacctgggcgatgacgaaaatgtgcaggaactgtactacattagcctgcattttcgcctgctgcgccagaatggctacaaaatcagcgcggatgtctttaatagctttaaggacagcaatggcaattttaaaagctttctgaagcgcgatattcgcggcatgctgagcctgtacgaagccgcgcatctgcgcgttcacggcgaaaatatcctgaatgaagccctgacctttacggtgacccacctggaaagctttacgagccagagcaatacgcagctggcggcccaggttaatcgtgccctgaatcgcccgattcgcaaaagcctgccccgcctggaagcgaagcattacatgccgatctaccagaaagatcccagccacaataaggacctgctgacgtttgcgatgctggattttaatattctgcagaaacagcaccaggaagaactgcgcgatatcgtgcgttggtggaaaaattttgacgtcccgaataagctgccctttattcgcgaccgcgttgtggaaggctacttttggatcctgggcgtctactttgaaccgaagtttctgctggcccgcaaaattctgaccaaggttatcagcatggccagcattatcgatgacatttacgatgcgtacggcacgatcgaagaactggaactgtttgccaccgcgattgaacgctgggatctgagcgcgatcgacctgctgcccgaatacatgaaactgtgttactgcgccctgctggatgcgtacagcgaatttgaaaaagacctggccagcaagggcattctgtacggcctgccgtttgcgaaagaaagcatgaagatcctggtgcgcagctacattatcgaagcccgctggtgtgatcagcagtacgttcccacgatggaagaatacatgcgtgtggccctgctgagctgtggttacctgctgctgagcacgagcagctttctgggcatggaagacattgttaccaaagaagcctttgaatgggtcagcggcaatccgaagattgttcaggcgagcagcattatctgtcgcctgatggatgacatcgtgagccataaatttgaacagcagcgcggtcatgttgccagcgccgtggaatgctacatgaagcagcatggcgtgagcgaagaagaagccgtgaaagtctttcgcgaaaaggtcggcaatgcgtggaaagatatcaatgaagaactgatgcgcccgcccgttgttcccatgcctctgctggaacgcgtcctgaatctggcccgcctgatggatgttctgtaccagaataatgacagctacaccaatccgcacctgatgaaggaccatgttgccgccctgctgaaagaccctgtgttttttgaggactaa

SEQ ID NO: 107 - protein, 565 aa, Citrus unshiu
MLFQVSASPNKVIRINAEKESTRRSANFDPTIWGDYFLSYTGDFKESGDASVKHQELKKEIRTMLRADINKPTQTKLDLIDDIQRLGVSYHFESEIDEILRKMHEANQDCDLGDDENVQELYYISLHFRLLRQNGYKISADVFNSFKDSNGNFKSFLKRDIRGMLSLYEAAHLRVHGENILNEALTFTVTHLESFTSQSNTQLAAQVNRALNRPIRKSLPRLEAKHYMPIYQKDPSHNKDLLTFAMLDFNILQKQHQEELRDIVRWWKNFDVPNKLPFIRDRVVEGYFWILGVYFEPKFLLARKILTKVISMASIIDDIYDAYGTIEELELFATAIERWDLSAIDLLPEYMKLCYCALLDAYSEFEKDLASKGILYGLPFAKESMKILVRSYIIEARWCDQQYVPTMEEYMRVALLSCGYLLLSTSSFLGMEDIVTKEAFEWVSGNPKIVQASSIICRLMDDIVSHKFEQQRGHVASAVECYMKQHGVSEEEAVKVFREKVGNAWKDINEELMRPPVVPMPLLERVLNLARLMDVLYQNNDSYTNPHLMKDHVAALLKDPVFFED

SEQ ID NO: 108 - DNA, 1746 bp, Artificial Sequence
  DNA having modified codons, which encodes linalool synthase gene derived from Citrus unshiu (Cu2LINS)
atggcgtttagcagcaaggacatcagtagcgacagcagtcacattcattttatcccgaagcacatcagtaaggttggtaatcgtaacctgaataatattaatagcctgctgccgaacaacaaaaagggcagcatcaacgataacatcggcgtcagcgcccgcctgaaacgctttacctaccccagcgaacatagcagcaactttaacgatgacatccatatcaagcacgccaaaaagctggaagttattaaacacattctgatcaagctgggcgatgacgatagctttgaaggcctggcgatgattgacgttgtgcagcgcctgggcatcgactactactttcaggatgaaattgaactgatcctgcgtcgccagtacagcattttctttacggacggcgatcgctacaatgatctgcaggaagttgcgctgcgttttcgtctgctgcgtcagcagggctactacgtgagcgcggacgtctttaatcgctttcgcaacaaagaaggcgaatttaagcagaacatcagcgaagatatcaatggcctgatgagcctgtacgaagcgagccagctgagcatcggcggcgaagatggcctggatgaagccggccattttagcgccacccacctggcgaattacgatctggcgggcgtcgttgaacatctgctgctgtacccgtaccgcaaaagcctgagccccgccaagaatttctttcacggcaattttcagggcagcgaatacatttggatcctggacctgcaggaactggcgaatatggattttaaactggtgcagagcctgcatcagaaggaaattgtccagatcagcagttggtggcgcgaactgggcctggcgaaaaagctggaatttgcccgcgaacagccggttaaatggtacgtttggagcatggcctgttttaccgacccgaatctgagctggcagcgcattgaactgacgaaacccatcagctttgtttacatcatcgacgatatcttttacgtgtgtggtgccctggatgccctgaccctgtttacggaaccgattaatcgctgggatctgggcgacatcgatcagctgcccgaatacatgaagatttgttttaaggcgctgaacgatatcaccaatgaaatcagcaaacagggcgtgcagcgcagcatgggcattaccctgtgtacgccgctgcgtaagggcgttggcgaagtgctgtgcaatgcctttctgatcgaagccaaatggtttgcgagcggccatctgcccaaggcggaagaatacctggaaaatggcattgtcagcagcggcgttcatctggtgctggtccacattttctttctgctgggccacggcatcaccaatgaaacggtccagctgattgatagcaatccgcccatcgtcagcagcgttgcgacgattctgcgcatctgggacgatctgggcagcgccaaagacgaaaatcagggcggcaaggatggcagctacatttactactacatgatggaacaccgcgacctgaccgccgaagatgcgcataaacacgcgatggacaagatcagcgatgcctggaaacgcctgaataaggaatgtctgagcccgaatccctttagcgccagctttacgcgcgcgagctttaattgcgcccgcatggtgccgctgatgtacagctacgacgatagccagcgcctgcccagcctggaagaatacattaagagcagtctgtttgacaatctgcctacgcagggtgtttactaa

SEQ ID NO: 109 - protein, 581 aa, Citrus unshiu
MAFSSKDISSDSSHIHFIPKHISKVGNRNLNNINSLLPNNKKGSINDNIGVSARLKRFTYPSEHSSNFNDDIHIKHAKKLEVIKHILIKLGDDDSFEGLAMIDVVQRLGIDYYFQDEIELILRRQYSIFFTDGDRYNDLQEVALRFRLLRQQGYYVSADVFNRFRNKEGEFKQNISEDINGLMSLYEASQLSIGGEDGLDEAGHFSATHLANYDLAGVVEHLLLYPYRKSLSPAKNFFHGNFQGSEYIWILDLQELANMDFKLVQSLHQKEIVQISSWWRELGLAKKLEFAREQPVKWYVWSMACFTDPNLSWQRIELTKPISFVYIIDDIFYVCGALDALTLFTEPINRWDLGDIDQLPEYMKICFKALNDITNEISKQGVQRSMGITLCTPLRKGVGEVLCNAFLIEAKWFASGHLPKAEEYLENGIVSSGVHLVLVHIFFLLGHGITNETVQLIDSNPPIVSSVATILRIWDDLGSAKDENQGGKDGSYIYYYMMEHRDLTAEDAHKHAMDKISDAWKRLNKECLSPNPFSASFTRASFNCARMVPLMYSYDDSQRLPSLEEYIKSSLFDNLPTQGVY

SEQ ID NO: 110 - DNA, 1767 bp, Artificial Sequence
  DNA having modified codons, which encodes linalool synthase gene derived from Citrus unshiu (Cu3LINS)
atggcgtttagtagcagtagccgtgcgaagctgagtgcgacgagtcacattagcaaagcccctgataagattagcaagacgagccgtccgagcctgattgaatttacgccgagccccaccatttaccagaaaggctgtatcacgagcgataataccgtcgcgagcccgcccctgaagcattttacgcacaccacgcgccatcccagctttttcgatcacgacattcaggtcgaacatagccgcaagctgaaggaatttaagcatatctttagcctggttggcggcaatagctttgaaggcctggtgatgattgatgccgtccagcgcctgcgcatcgaatacctgtttaaggacgaaattgaagaaatcctgcagcgccagtacattatcagcagcacgtgtggtggccatctgcacgatctgcaggaagttgcgctgcgctttcgcctgctgcgccaggaaggctactacgtgccggccgatatgtttaacaactttcgcatcaaagaaggccgctttagccgcattaatgtcagcgaagacatcggcaccctgatggaagtttacgaagcgagccagctgagcatcgccggcgaagaaggcctggatgaagccggccactttagcgcgaagatgctgaatgaatgcatgacgcatctggaccattaccacgccctggcgatcggcaataccctgcgccatccgtaccacaaaagcctgccccgctttatggccaaggatgtgtttctgagcaattttcagggcgaacgccgcctgcacgtgctgaaggaaatcgcgaaaaaggactttaacatggtccaggccctgcatcagaaggaaatcgttcaggtgacgaaatggtggaaggatctgggcctgaccaaaaagctgccgtttgcgcgcgaccagcccctgaaatggtacatttggagcatggcctgtctgacggatccgagcctgagcgaacagcgcgtggaactgaccaagcccattagcctgatctacattatcgatgacatctttgatgtctacggcacgctggacgaactgattctgtttaccgaaacgatcacgcgttgggacctggcggccatgggtcagctgccggaatacatgaaaatttgttttaaggcgctggatgacattacgaatgaaatcagctgcaaagtttacaaaaagcacggctacaatccggtgcagagcctgcgcaatgcgtggaccagcctgtgcaaagcctttctggttgaagccaagtggtttgcgagcggccatatgcccgaagccgaagaatacctgcgcaatggcatcgaaagcagcggcgtccatgttgccctggcgcactttttctttctgctgggccacggcattacgaaagaaaccgtggaactgatcgatggcaatcccgcgattatcagcagcacggccaccattctgcgtctgtgggatgacctgggtagcgccaaagatgaaaatcaggaaggcaaggacggcagctacatccactactacatgaaagaacatcgctacagcgccgcggaagaagcccagaaaagcgcgattaataagatcagcgacgcctggaaacgcctgaataaggaatgtctgtgcccgaatccctttagcgccagctttacgcgtgccagcctgaatctggcccgtatggttccgctgatgtacagctacgatgacaatcagcgcctgcccagcctggaacattacattaagagcctgctgtttgagagcgtgcctacggagggcgtctactaa

SEQ ID NO: 111 - protein, 588 aa, Citrus unshiu
MAFSSSSRAKLSATSHISKAPDKISKTSRPSLIEFTPSPTIYQKGCITSDNTVASPPLKHFTHTTRHPSFFDHDIQVEHSRKLKEFKHIFSLVGGNSFEGLVMIDAVQRLRIEYLFKDEIEEILQRQYIISSTCGGHLHDLQEVALRFRLLRQEGYYVPADMFNNFRIKEGRFSRINVSEDIGTLMEVYEASQLSIAGEEGLDEAGHFSAKMLNECMTHLDHYHALAIGNTLRHPYHKSLPRFMAKDVFLSNFQGERRLHVLKEIAKKDFNMVQALHQKEIVQVTKWWKDLGLTKKLPFARDQPLKWYIWSMACLTDPSLSEQRVELTKPISLIYIIDDIFDVYGTLDELILFTETITRWDLAAMGQLPEYMKICFKALDDITNEISCKVYKKHGYNPVQSLRNAWTSLCKAFLVEAKWFASGHMPEAEEYLRNGIESSGVHVALAHFFFLLGHGITKETVELIDGNPAIISSTATILRLWDDLGSAKDENQEGKDGSYIHYYMKEHRYSAAEEAQKSAINKISDAWKRLNKECLCPNPFSASFTRASLNLARMVPLMYSYDDNQRLPSLEHYIKSLLFESVPTEGVY

SEQ ID NO: 112 - DNA, 1704 bp, Artificial Sequence
  DNA having modified codons, which encodes linalool synthase gene derived from Malus domestica (MdLINS)
atggagtttagcattagccagagtagttttgcgaccagtagcagcacgcccgccgcccctgagcacctgagcagccagaagtggagtattcccgaagatcatagcctgctgagcaccccgctgaaaccgctgaatagcaaaaccaagtacacgagcagcaaggacggcatcatttgttttcagaacgaacagaagctggatgacctgcgccatgcgctgattaaggttggcggcgaagccgtggaaagcctggatatgatcgacgcggttcagcgcctgggcctggattaccactttgaagaagaaattgaccagatcctgcagaaacagcatattatcagcagcacgaccgcccatggtgcccatcaccccaccgatctgcatgaagttgccctgcgttttcgtctgctgcgtcagcacggctactttgtgagcgatgacgtctttaacaactttaagaaccgcgaaggcaactttaatcagatgctgcgcgaagacattaagggcctgatgagcctgtacgaagcgagccagctgagcatcgaaggcgaagttgtgctggaagaagccggcaaatttagcggccattttctgaatagcagcctgagccacctggatcatcaccaggcgcgcgtcgttggcaataccctgcgcaatccccatcacaaaagcctggccccgtttatggcgaagaatttctttgtcagcagctttcagggcacgaataatcgctggctgaatattctgcagaccgtggcgaaaacggatctgaatatggtccagagcctgcatcagaaggaagtcgcccaggttagcaaatggtggaaggaactgggcctgtgtaaagaactgaagtttgcgcgcgatcagcccattaaatggtacatctggagcatggcctgcctgaccaatcccaatctgagcgacgaacgcatcgaactgacgaagccgattagctttatctacctgattgatgacatctttgatgtgtacggcaccctggacgaactgaccctgtttacggaagtggtcaatcgctgggaaattggcagcatcgaacacctgccggattacatgaaaatttgttttaaggcgctgtacgacatgaccaatgaaatcagctgcaaagtctaccagaagcatggctggaatcccctgcacagcctgaaaaagacgtgggccagcctgtgcaatgcgtttctggttgaagccaaatggtttaagagcggccatctgccgatggccgaagaatacctgaaaaatggcattatcagcagcggcgtcaatgttgtgatggttcacattttctttctgctgggcgaaggcatcaccaatcagagcgtggaatttctgaatggcaccccggcgattatcagcagcaccgcggccattctgcgcctgtgggatgacctgggtagcgccaaggatgaaaatcaggacggcgatgacggcagctacgtcaaactgtacctgaatgaacatcagggcaagaccatggaagaagcccaggaacacgttacgaatatgatcagcgaagaatggaaaaagctgaataaagaactggtgagccccaatcccctgcccgcggcctttaccaaggccagcctgaatctggcccgcatggttccgctgatgtacagctacgacgataatcagtgtctgccgagtctggatgagtacatgaagagtatgctgcacgcctaa

SEQ ID NO: 113 - protein, 567 aa, Malus domestica
MEFSISQSSFATSSSTPAAPEHLSSQKWSIPEDHSLLSTPLKPLNSKTKYTSSKDGIICFQNEQKLDDLRHALIKVGGEAVESLDMIDAVQRLGLDYHFEEEIDQILQKQHIISSTTAHGAHHPTDLHEVALRFRLLRQHGYFVSDDVFNNFKNREGNFNQMLREDIKGLMSLYEASQLSIEGEVVLEEAGKFSGHFLNSSLSHLDHHQARVVGNTLRNPHHKSLAPFMAKNFFVSSFQGTNNRWLNILQTVAKTDLNMVQSLHQKEVAQVSKWWKELGLCKELKFARDQPIKWYIWSMACLTNPNLSDERIELTKPISFIYLIDDIFDVYGTLDELTLFTEVVNRWEIGSIEHLPDYMKICFKALYDMTNEISCKVYQKHGWNPLHSLKKTWASLCNAFLVEAKWFKSGHLPMAEEYLKNGIISSGVNVVMVHIFFLLGEGITNQSVEFLNGTPAIISSTAAILRLWDDLGSAKDENQDGDDGSYVKLYLNEHQGKTMEEAQEHVTNMISEEWKKLNKELVSPNPLPAAFTKASLNLARMVPLMYSYDDNQCLPSLDEYMKSMLHA

SEQ ID NO: 114 - DNA, 1824 bp, Artificial Sequence
  DNA having modified codons, which encodes linalool synthase gene derived from Perilla frutescens var. crispa (PfLINS)
atgtatagcctgcgtatttatgtggcgattatgaaaaagcccagtgcgaagcatgttgacaatgtggacaagaaagcgagtaagcctagctggcgcgttagcctgagcagcagcgcgggcctgcgtgccagcagcagcctgcagctggatgtgaaaaagccggcggatgatgaaatcctgacggcccgccgcagcggtaattaccagcccagcctgtgggactttaattacctgcagagcctgaataccacgcagtacaaagaagtgcgccatctgaagcgcgaagcggaactgattgaacaggtcaaaatgctgctggaagaagaaatggaagccgtccagcagctggaactggttgatgacctgaagaatctgggcctgagctactttttcgaagatcagattaaacagatcctgacgtttatctacaacgaacataagtgttttcacagcaatagcattatcgaagcggaagaaattcgcgacctgtactttacggccctgggttttcgtctgctgcgtcagcatggctttcaggttagccaggaagtgtttgattgctttaagaatgaagaaggcagcgactttaaagcccgtctgggtgatgacaccaagggcctgctgcagctgtacgaagccagctttctgctgcgcgaaggcgaagatacgctggaactggcccgccagtacgcgaccaaatttctgcagaaaaaggtggaccacgaactgatcgatgacaataatctgctgagctggattctgcatagcctggaaatcccgctgcactggcgcattcagcgcctggaagcgcgctggtttctggatcgctacgccacgcgtcgcgacatgaatcagattatcctggaactggcgaaactggattttaatattatccaggccacgcagcaggaagaactgaaagacctgagccgttggtggaagagcacctgtctggcggaaaaactgccgtttgtgcgcgatcgcctggtcgaaagctacttttgggccattgcgctgtttgaaccccatcagtacggctaccaccgcaaagtcgccgcgaagattatcaccctgatcacgagcctggatgacgtttacgatatttacggcaccctggacgaactgcagctgtttacggatgcgatccagcgctgggacaccgaaagcattagccgcctgccctactacatgcagctgttttacatggttctgtacaattttgtgagcgaactggcctacgatggcctgaaagaaaagggctttattaccattccctacctgcagcgtagctgggcggacctggtggaagcgtacctgaaagaagccaagtggttttacaatggctacgtccccagcatggaagaatacctgaataatgcgtacattagcattggtgccaccccggtcatcagccaggttttctttaccctggccacgagcattgataaacccgtcatcgacagcctgtacgaataccatcgcattctgcgtctgagcggtatgctggttcgcctgcccgatgacctgggtacgagcccctttgaaatgaaacgcggcgatgttccgaaggcgatccagctgtacatgaaagaacgcaatgcgacggaaatcgaagcccaggaacacgttcgctttctgattcgcgaagcctggaaggaaatgaataccgttaccacggccgcggattgcccctttaccgatgacctggttgcggccacccgtaatctgggtcgtgccgcgcagtttatgtacctggatggcgacggtaaccacagtcagctgcaccagcgtatcgcctgcctgctgtttgaaccctatgcctaa

SEQ ID NO: 115 - protein, 607 aa, Perilla frutescens var.crispa
MYSLRIYVAIMKKPSAKHVDNVDKKASKPSWRVSLSSSAGLRASSSLQLDVKKPADDEILTARRSGNYQPSLWDFNYLQSLNTTQYKEVRHLKREAELIEQVKMLLEEEMEAVQQLELVDDLKNLGLSYFFEDQIKQILTFIYNEHKCFHSNSIIEAEEIRDLYFTALGFRLLRQHGFQVSQEVFDCFKNEEGSDFKARLGDDTKGLLQLYEASFLLREGEDTLELARQYATKFLQKKVDHELIDDNNLLSWILHSLEIPLHWRIQRLEARWFLDRYATRRDMNQIILELAKLDFNIIQATQQEELKDLSRWWKSTCLAEKLPFVRDRLVESYFWAIALFEPHQYGYHRKVAAKIITLITSLDDVYDIYGTLDELQLFTDAIQRWDTESISRLPYYMQLFYMVLYNFVSELAYDGLKEKGFITIPYLQRSWADLVEAYLKEAKWFYNGYVPSMEEYLNNAYISIGATPVISQVFFTLATSIDKPVIDSLYEYHRILRLSGMLVRLPDDLGTSPFEMKRGDVPKAIQLYMKERNATEIEAQEHVRFLIREAWKEMNTVTTAADCPFTDDLVAATRNLGRAAQFMYLDGDGNHSQLHQRIACLLFEPYA

SEQ ID NO: 116 - DNA, 1734 bp, Artificial Sequence
  DNA having modified codons, which encodes linalool synthase gene derived from Vitis vinifera (Vv1LINS)
atgggttttagtcctgccttttatgcgtgtagtatccctcccgttggtccgaacaagtttaccgagctgggtcagagcaagtttaacaatgttgtgctggttccgaccgcccagaaatggagcattgcgcatgatcacacgctggtgtacaaacccctgcgcaagcataatcaccagagccagcatctgagctttaccgatgaattttacattaagcacgcgcagcgcctggacgaaatccgcaatgtctttagcgaagttggcgaagacacgctggaaggcctgatgatgattgatgccatccagcgcctgggcatcgactaccattttaaagaagaaatcgaagccgtcctgcagcgccagtacatgaaggcgagcacccacggcgaaagcattcaggatctgtacgaagttgccctgcgttttcgtctgctgcgtcaggaaggctaccatgtgccggccgatgtctttaacaactttaagaacaaggaaggcaaatttaagcagaatctgagcaaagacatcaagggcctgctggccctgtacgaagcgagccagctgagcattgaaggcgaagatatcctggaagaagcccagcgctttagcagcaccctgctgaatgcgggcctggaacacctgaatcatcacgaagccaccgtcgttggccatacgctggaacacccgcatcacaaaagcctgccccgctttatggcgaaaagctttctgaaggattttcagggccccaatggctggctgacggtcctgcaggaactggccaaagcggactttaatatggttcagagcattcatcagcaggaactgctgcagatcagcaaatggtggcaggatcgcggcctggccgaagaactgaaatttgcgcgcgaccagccgctgaagtggcacatgtggccgatggccgttctgcccgaccctagcctgagcgaacagcgtgtggaactgaccaaaccgattagcatgatctacatcatcgatgacatctttgatgtgcatggcacgctggacgaactgaccctgtttacggaagccgtcaatcgctgggacattgccgcgtttgaaaccctgcccaactacatgaagatttgttttaagaccctggatgaaatcacgaacgaaatcagcaacaaggtttacaaggaacacggctggaatccggttgatagcctgcgcaaaacgtgggtgagcctgtgcaatgcgtttctggtcgaagccaagtggtttgcgagcggccatgtgcccaaagcccacgaatacctgaagaatggcgttattagcagcggcgtgcatgtggtcctggtccacctgtttttcctgctgggccatggcatcacccgcggcaatgttgacctggtggatgactttccgagcattatcagcagcaccgcggccattctgcgtctgtgggatgacctgggtagcgcgaaagatgaaaatcaggatggccatgacggcagctacattgaatgttacatcaaggaacaccagggcagcagcatggaaaatgcccgccagaatgttacgtacatgattagcgatctgtggaaacgcctgaataaggaatgcctgagccagcacccgtttagcaccagctttacgaaaggcagcctgaatatcgcccgcatggtgcccctgatgtacagctacgatgacaatcagagcctgccccatctggaggagcacatgaagagtctgctgtttgaagcgtttcccctgtaa

SEQ ID NO: 117 - protein, 577 aa, Vitis vinifera
MGFSPAFYACSIPPVGPNKFTELGQSKFNNVVLVPTAQKWSIAHDHTLVYKPLRKHNHQSQHLSFTDEFYIKHAQRLDEIRNVFSEVGEDTLEGLMMIDAIQRLGIDYHFKEEIEAVLQRQYMKASTHGESIQDLYEVALRFRLLRQEGYHVPADVFNNFKNKEGKFKQNLSKDIKGLLALYEASQLSIEGEDILEEAQRFSSTLLNAGLEHLNHHEATVVGHTLEHPHHKSLPRFMAKSFLKDFQGPNGWLTVLQELAKADFNMVQSIHQQELLQISKWWQDRGLAEELKFARDQPLKWHMWPMAVLPDPSLSEQRVELTKPISMIYIIDDIFDVHGTLDELTLFTEAVNRWDIAAFETLPNYMKICFKTLDEITNEISNKVYKEHGWNPVDSLRKTWVSLCNAFLVEAKWFASGHVPKAHEYLKNGVISSGVHVVLVHLFFLLGHGITRGNVDLVDDFPSIISSTAAILRLWDDLGSAKDENQDGHDGSYIECYIKEHQGSSMENARQNVTYMISDLWKRLNKECLSQHPFSTSFTKGSLNIARMVPLMYSYDDNQSLPHLEEHMKSLLFEAFPL

SEQ ID NO: 118 - DNA, 1809 bp, Artificial Sequence
  DNA having modified codons, which encodes linalool synthase gene derived from Vitis vinifera (Vv2LINS)
atggaactgaccctgacgagtctgagcccgctggcgtatggtgccctgaactgccgtaagaactttgcgatggcgagtccccgtatgcgcattaagcagggccgcagcgaactgccgaatctgacgattaccagcaaaatcgacgaactgcaggtgaccgaacgccgcagcgcgaattaccacccgagcatttgggatcccaaatttatcgaaagcctgagcacgccctacaccaatgaaggctacagcaatcagctggaagatctgaaagaagaagccaagcgcgtcattaaagatgcgcgcgacacgagcagccgcctggaatttatcgacagcatgcagcgcctgggcgtggcctaccatctggaagaagaaattaaggaagcgatcgatctggtccacctggatgacaccacgaccgatgacctgagcaccacggccctgcgttttcgtctgctgcgtcagcatggttacccggtcagcagcgaagtttttgatcagtttcgcagcaaagatggccgctttatggacggcattagccaggatattgcgggtcctctgagcctgtacgaagccagccatctgggcgttgaaggcgaagatgacctggaagaagcccgccgctttagcaccatccacctgaagagcctggtgggcaatctggaaagcgatctggcggaccaggtgcagcagagcctggaagtccccctgcactggcgtatgcctcgtctggaagcccgcaattttattgacatctaccagcgtcgcaataccaagaatagcgccctgctggaactggcgaaactggattacaatctggttcagagcagctaccagacggaactgaaagaactgacgcgttggtggaccgacctgggctttaaagaaaagctgagctttagccgcgatcgcctgatggaaaattacctgtggagcatgggcattgcgccggaaccccattttagcaagagccgcatcggcctgaccaaatttatttgtatcctgacggccattgatgacatgtacgacatctacggcagcccggatgaactgcgccgctttaccgacgccgtcaatcgctgggatacggaagcgctggttgatctgcccgactacatgaagatttgttacctggccatgtttaactttgcgaatgaaatggcctacgatgcgctgcgcgatcatgacctgtacatcctgccgtacctgaagagccagtggctgaatctgtgcaccagctacagcatggaagcccagtggttttacaatggctacaaaccgagcattgatgaatacctgagcaatgcctggaccagcgttggcggcccggcggccatggtgcacgcctactttctgatgggctgtgcgacgaagggcaatctgaataattgcctggacaatgcgagcaatctgctgtactggagcagcctgatcacgcgtctgagcgatgacctgggtacgagcctggcggaaattgcccgcggcgatgtcgccaagagcatccagtgttacatgattgaaaaatgcatcagcgaagaacaggcgcgcgaccaggttgaaaagctgattcgctacagctggaaaaagctgaatgaagccagcacggatagcagcctgccgaaaagcctgatcaatagcagcctgaatatggcccgcagcgcgcagtgcatttttcagtttggtgatggtattggtacgagcgttggcgtgaccaaggatcgcctgacgagctttattatcaaacccattctgattgaaccgagcattaagccctacctggatggcatgaagatgagtaaccgccgctaa

SEQ ID NO: 119 - protein, 602 aa, Vitis vinifera
MELTLTSLSPLAYGALNCRKNFAMASPRMRIKQGRSELPNLTITSKIDELQVTERRSANYHPSIWDPKFIESLSTPYTNEGYSNQLEDLKEEAKRVIKDARDTSSRLEFIDSMQRLGVAYHLEEEIKEAIDLVHLDDTTTDDLSTTALRFRLLRQHGYPVSSEVFDQFRSKDGRFMDGISQDIAGPLSLYEASHLGVEGEDDLEEARRFSTIHLKSLVGNLESDLADQVQQSLEVPLHWRMPRLEARNFIDIYQRRNTKNSALLELAKLDYNLVQSSYQTELKELTRWWTDLGFKEKLSFSRDRLMENYLWSMGIAPEPHFSKSRIGLTKFICILTAIDDMYDIYGSPDELRRFTDAVNRWDTEALVDLPDYMKICYLAMFNFANEMAYDALRDHDLYILPYLKSQWLNLCTSYSMEAQWFYNGYKPSIDEYLSNAWTSVGGPAAMVHAYFLMGCATKGNLNNCLDNASNLLYWSSLITRLSDDLGTSLAEIARGDVAKSIQCYMIEKCISEEQARDQVEKLIRYSWKKLNEASTDSSLPKSLINSSLNMARSAQCIFQFGDGIGTSVGVTKDRLTSFIIKPILIEPSIKPYLDGMKMSNRR

SEQ ID NO: 120 - DNA, 1695 bp, Artificial Sequence
  DNA having modified codons, which encodes linalool synthase gene derived from Lavandula angustifolia (LaLINS)
atgagtatcaacattaacatgcccgccgccgccgttctgcgtccgtttcgttgtagtcagctgcacgtcgatgagacccgccgtagtggcaattaccgcccgagcgcctgggacagcaattacatccagagcctgaatagccagtacaaggaaaagaaatgtctgacgcgcctggaaggcctgattgaacaggttaaagaactgaagggcaccaaaatggaagcggtgcagcagctggaactgatcgatgacagccagaatctgggcctgagctactactttcaggataagatcaagcatatcctgaacctgatctacaacgaccacaagtacttttacgatagcgaagccgaaggcatggacctgtactttacggcgctgggctttcgcctgtttcgccagcatggctttaaggttagccaggaagtgtttgatcgctttaagaacgaaaacggcacctactttaagcacgatgacacgaaaggcctgctgcagctgtacgaagccagctttctggttcgcgaaggcgaagaaaccctggaacaggcccgcgaatttgcgacgaagagcctgcagcgcaaactggatgaagacggcgatggcattgatgcgaatatcgaaagctggattcgccatagcctggaaattccgctgcattggcgtgcccagcgtctggaagcccgttggtttctggatgcctacgcccgccgccctgatatgaatcccgtcatctttgaactggccaagctgaactttaacatcgttcaggccacgcagcaggaagaactgaaagccctgagccgttggtggagcagcctgggcctggccgaaaaactgccctttgtgcgcgaccgcctggtcgaaagttacttttgggccatcccgctgtttgaaccccatcagtacggctaccagcgcaaggtggcgaccaaaattatcaccctgatcacgagcctggatgacgtctacgacatttacggcaccctggatgaactgcagctgtttacgaacctgtttgaacgctgggataatgccagcatcggccgcctgccggaatacctgcagctgttttactttgccattcacaattttgtcagcgaagttgcgtacgacatcctgaaagaaaagggctttaccagcattgtgtacctgcagcgcagctgggtcgatctgctgaagggctacctgaaggaagccaaatggtacaatagcggctacaccccgagcctggaagaatactttgataatgcctttatgacgattggtgcccctccggtgctgagccaggcctactttaccctgggcagcagcatggaaaaacccattatcgaaagcatgtacgaatacgacaatatcctgcgcgttagcggtatgctggttcgcctgcccgatgacctgggtacgagcagctttgaaatggaacgcggcgatgtccccaagagcgttcagctgtacatgaaagaaaccaatgccacggaagaagaagccgtggaacatgtccgctttctgaatcgcgaagcctggaaaaagatgaatacggccgaagcggccggtgacagccccctggtcagcgatgttgttgcggttgcggccaatctgggtcgtgccgcgcagtttatgtactttgacggcgatggtaaccagagtagcctgcagcagtggattgtcagtatgctgtttgaaccgtatgcctaa

SEQ ID NO: 121 - protein, 564 aa, Lavandula angustifolia
MSININMPAAAVLRPFRCSQLHVDETRRSGNYRPSAWDSNYIQSLNSQYKEKKCLTRLEGLIEQVKELKGTKMEAVQQLELIDDSQNLGLSYYFQDKIKHILNLIYNDHKYFYDSEAEGMDLYFTALGFRLFRQHGFKVSQEVFDRFKNENGTYFKHDDTKGLLQLYEASFLVREGEETLEQAREFATKSLQRKLDEDGDGIDANIESWIRHSLEIPLHWRAQRLEARWFLDAYARRPDMNPVIFELAKLNFNIVQATQQEELKALSRWWSSLGLAEKLPFVRDRLVESYFWAIPLFEPHQYGYQRKVATKIITLITSLDDVYDIYGTLDELQLFTNLFERWDNASIGRLPEYLQLFYFAIHNFVSEVAYDILKEKGFTSIVYLQRSWVDLLKGYLKEAKWYNSGYTPSLEEYFDNAFMTIGAPPVLSQAYFTLGSSMEKPIIESMYEYDNILRVSGMLVRLPDDLGTSSFEMERGDVPKSVQLYMKETNATEEEAVEHVRFLNREAWKKMNTAEAAGDSPLVSDVVAVAANLGRAAQFMYFDGDGNQSSLQQWIVSMLFEPYA

SEQ ID NO: 122 - DNA, 1821 bp, Artificial Sequence
  DNA having modified codons, which encodes linalool synthase gene derived from Mentha citrata (McLINS)
atgtgtaccatcattagcgtcaatcatcatcatgtcgccatcctgagcaagccgaaggtcaagctgtttcataccaagaataagcgcagcgccagcatcaatctgccgtggagcctgagccctagcagcagcgcggccagccgcccgattagctgtagcatcagcagcaaactgtacaccatcagcagcgcccaggaagaaacgcgccgcagcggcaattaccatcccagcgtttgggattttgactttattcagagcctggataccgaccactacaaggaagaaaaacagctggaacgcgaagaagaactgatcatggaagtgaaaaagctgctgggcgcgaagatggaagccacgaaacagctggaactgattgatgacctgcagaatctgggcctgagctactttttccgcgacgaaatcaagaacatcctgaacagcatctacaagatctttcagaacaacaatagcaccaaggttggcgatctgcattttacgagcctgggttttcgtctgctgcgtcagcacggctttaatgttagccagggcgtgtttgattgctttaaaaatgaacatggcagcgactttgaaaagaccctgatcggcgaagatacgaaaggcgtgctgcagctgtacgaagcgagctttctgctgcgcgaaggcgaagataccctggaagtcgcccgcaaatttagcacggaatttctggaagaaaaactgaaggcgggcattgatggcgacaatctgagcagcagcattggccatagcctggaaatcccgctgcactggcgcattcagcgcctggaagaacgctggtttctggatgcctacagccgtcgcaaggacatgaatcccattatctttgaactggcgaaactggactttaatattatccaggccacccagcaggaagaactgaaggatctgagccgttggtggaatgacagcagcctgccgcagaaactgccctttgtccgcgatcgcctggttgaaagctactactgggcgctgggcctgtttgaagcccataagtttggctacgaacgcaagacggccgcgaaaattatcaccctgatcacggcgctggatgacgtgtacgatatttacggcaccctggacgaactgcagctgtttacgcacgtcattcgccgctgggacacggaaagcgccacccagctgccgtactacctgcagctgttttactttgtcctgtacaattttgtcagcgaagttgcgtaccatattctgaaagaagaaggctttattagcatcccctttctgcaccgcgcgtgggtggatctggtcgaaggctacctgcaggaagccaagtggtactacaccaaatacaccccgacgatggaagaatacctgaattacgccagcattaccattggtgccccggccgttattagccagatctactttatgctggcgaaaagcaaggaaaaaccggtgatcgaaagcttttacgaatacgacgaaattattcgtctgagcggtatgctggttcgcctgcccgatgacctgggtaccctgccctttgaaatgaagcgcggcgatgttgccaaaagcattcagatctacatgaaggaacagaatgcgacgcgcgaagaagccgaagaacacgtgcgctttatgattcgcgaagcgtggaaagaaatgaataccacgatggccgcgaatagcgatctgcgcggcgacgttgtgatggcggccgccaatctgggtcgtgatgcccagtttatgtacctggatggcgacggtaatcatagtcagctgcagcaccgcatcgccaatctgctgtttaagccctacgtctaa

SEQ ID NO: 123 - protein, 606 aa, Mentha citrata
MCTIISVNHHHVAILSKPKVKLFHTKNKRSASINLPWSLSPSSSAASRPISCSISSKLYTISSAQEETRRSGNYHPSVWDFDFIQSLDTDHYKEEKQLEREEELIMEVKKLLGAKMEATKQLELIDDLQNLGLSYFFRDEIKNILNSIYKIFQNNNSTKVGDLHFTSLGFRLLRQHGFNVSQGVFDCFKNEHGSDFEKTLIGEDTKGVLQLYEASFLLREGEDTLEVARKFSTEFLEEKLKAGIDGDNLSSSIGHSLEIPLHWRIQRLEERWFLDAYSRRKDMNPIIFELAKLDFNIIQATQQEELKDLSRWWNDSSLPQKLPFVRDRLVESYYWALGLFEAHKFGYERKTAAKIITLITALDDVYDIYGTLDELQLFTHVIRRWDTESATQLPYYLQLFYFVLYNFVSEVAYHILKEEGFISIPFLHRAWVDLVEGYLQEAKWYYTKYTPTMEEYLNYASITIGAPAVISQIYFMLAKSKEKPVIESFYEYDEIIRLSGMLVRLPDDLGTLPFEMKRGDVAKSIQIYMKEQNATREEAEEHVRFMIREAWKEMNTTMAANSDLRGDVVMAAANLGRDAQFMYLDGDGNHSQLQHRIANLLFKPYV

SEQ ID NO: 124 - DNA, 1608 bp, Artificial Sequence
  DNA having modified codons, which encodes linalool synthase gene derived from Ocimum basilicum (Ob1LINS)
atggcgagtgcggtccccctgagtagtacgcccctgattaacggcgacaatagtcccctgaaaaatacccaccagcatgttgaggagcgcagcagcaaacgtcgcgaatacctgctggaagaaaccgcgcgcaagctgcagcgcaatgacacggaaagcgttgaaaaactgaagctgattgataatatccagcgcctgggcattggctactactttgaagatgccattgatgcggtgctgcgcagcccctttagcgccgaagaagaagaagacctgtttaccgcggccctgcgttttcgtctgctgcgtcataatggcattcaggtcaccccggaaatctttctgaaatttaaggatgaacgcggcgaatttgacgaaagcgatacgctgggcctgctgagcctgtacgaagcgagcaatctgggcgtgaccggcgaagaaatcctggaagaagcgatggaatttgcggaaccccgtctgcgccgcagcctgagcgaactggccgcgcccctgcgcagcgaagtcgcccaggccctggatgttccccgtcacctgcgcatggcccgtctggaagcccgccgctttattgaacagtacggcaaacagagcgatcatgacggcgatctgctggaactggcgattctggactacaatcaggtccaggcccagcaccagagcgaactgaccgaaatcacgcgttggtggaaacagctgggcctggttgaaaaactgggttttggtcgcgatcgcgccctggaatgttttatgtggacgatgggcattctgccgcatcccaaatacagcagcagccgtattgaaagcgccaaggcggccgccctgctgtacgttattgatgacatctttgacacctacggcaaaatggatgaactgattctgtttacggacgcgatccgccgctgggatctggaagccatggaaggcctgcccgaatacatgaagatttgttacatggcgctgtacaataccacgaatgaaatttgctaccgcgttctgaaagataccggtcgtattgccctgccttacctgaagagcgtgtggattgaaaccatcgaagcgtacatggtcgaagttaaatggtttagcggcggcagcgcccccaagctggaagaatacattgaaaatggtgccagcaccgtgggtgcctacatggtgctggtccacctgtttttcctgatcggcgaaggcctgacccaccagaatgtcctgtttttcaaacagaagccgtaccacaaaccctttagcgccgcgggtcgtatttttcgtctgtgggatgacctgggcacgagccaggaagaagaagaacgcggcgatatggcgagcagcatccgcctgtttatgaaagaatacaagctgagcaccgtggaagaagcccgcagctgcgtcctggaagaaattagccgcctgtggaaagacctgaatgaaggcctgattagcatcaaagatgccctgccgctgaccattgttaaggtggcgctgaatatcgcccgcacgagccaggttgtgtacaagcatgaacagcacacctacatgctgagtgttgacaattatgtggaagccctgttttttacgcccctgctgagtagttaa

SEQ ID NO: 125 - protein, 535 aa, Ocimum basilicum
MASAVPLSSTPLINGDNSPLKNTHQHVEERSSKRREYLLEETARKLQRNDTESVEKLKLIDNIQRLGIGYYFEDAIDAVLRSPFSAEEEEDLFTAALRFRLLRHNGIQVTPEIFLKFKDERGEFDESDTLGLLSLYEASNLGVTGEEILEEAMEFAEPRLRRSLSELAAPLRSEVAQALDVPRHLRMARLEARRFIEQYGKQSDHDGDLLELAILDYNQVQAQHQSELTEITRWWKQLGLVEKLGFGRDRALECFMWTMGILPHPKYSSSRIESAKAAALLYVIDDIFDTYGKMDELILFTDAIRRWDLEAMEGLPEYMKICYMALYNTTNEICYRVLKDTGRIALPYLKSVWIETIEAYMVEVKWFSGGSAPKLEEYIENGASTVGAYMVLVHLFFLIGEGLTHQNVLFFKQKPYHKPFSAAGRIFRLWDDLGTSQEEEERGDMASSIRLFMKEYKLSTVEEARSCVLEEISRLWKDLNEGLISIKDALPLTIVKVALNIARTSQVVYKHEQHTYMLSVDNYVEALFFTPLLSS

SEQ ID NO: 126 - DNA, 2550 bp, Artificial Sequence
  DNA having modified codons, which encodes linalool synthase gene derived from Clarkia breweri (CbLINS)
atgcgtgagagcctgagcagtagcagtagcaatacccagaacctgtttctgagtacgagtccttacgatacggcgtggctggccctgattccgcatccccatcaccatcaccatcacggccgccctatgtttgaaaaatgtctgcagtggattctgcacaatcagaccccgcagggtttttgggcggccgcgggtgataatatcagcgacaccgatgacgatgtgacgctggactgtctgctgagcaccctggcctgcctggttgccctgaaacgttggcagctggccccggatatgattcataagggcctggaatttgtcaatcgcaataccgaacgcctggttatgaagcagaaaccgagcgacgtgccccgctggtttacgatcatgtttccggccatgctggaactggccggtgccagcagcctgcgcgtcgattttagcgaaaatctgaatcgcattctggttgaactgagccagaatcgcgacgatatcctgacccgcgaagaagtggatgaaaagaaacagtacagcccgctgctgctgtttctggaagccctgcccgcgcagagctacgacaatgatgttctgaaacagattatcgataagaatctgagcaatgacggcagcctgctgcagagccccagcgccacggcccgtgcctacatgatcaccggcaatacgcgctgtctgagctacctgcatagcctgacgaatagctgcagcaatggcggcgttccgagcttttaccccgtggacgatgacctgcacgacctggtcatggttaatcagctgacccgcagcggcctgacggaacatctgattccggaaatcgatcacctgctgctgaaggtgcagaaaaattacaagtacaaaaaggccagccccaaaagcctgtacagcattgcggccgaactgtaccgcgatagcctggcgttttggctgctgcgcgttaataatcattgggtgagcccgagcatcttttgttggtttctggatgacgatgaaattcgcgaccacatcgaaaccaattacgaagaatttgcggccgtgctgctgaatgtctaccgcgccacggatctgatgtttagcggcgaagttcagctggttgaagcccgcagctttgcgaccaaaaatctggaaaagattctggccaccggcaatatccataaaacgaatgcggacattagcagcagcctgcataagatgatcgaacatgaactgcgtgtgccttggaccgcccgtatggatcacgtcgaaaatcgcatttggatcgaagaaattgccagcagcgcgctgtggtttggcaaaagcagctacctgcgcctgagctgctttcataaaatgagcctgcagcagctggccgttaagaattacaccctgcgccagctggtctaccgcgacgaactggcggaagttgaacgctggagcaaagaacgcggcctgtgtgatatgggcttttgccgcgaaaagaccggctactgttactacgcctttgccgccagcacctgtctgccctggagcagcgatgtccgtctggttctgaccaaagcggccgttgtgatcacggtggcggacgatttctttgatgtcgaaggcagcatggttgatctggaaaaactgacggatgcggtccgccgctgggatgccgaaggcctgggcagccacagcaagacgatttttgaggccctggacgatctggtgaatgaagtccgcctgaaatgttttcagcagaatggccaggacatcaagaataatctgcagcagctgtggtacgaaacctttcatagctggctgatggaagcgaaatggggcaagggcctgaccagcaaaccgagcgtggatgtctacctgggcaatgccatgacgagcattgcggcccacaccatggttctgaccgccagctgtctgctgggtcccggttttccggtgcatcagctgtggagccagcgtcgccaccaggatatcaccagcctgctgatggtgctgacgcgcctgctgaatgacattcagagctacctgaaagaagaagatgaaggcaagatcaactacgtttggatgtacatgatcgaaaacaatcaggccagcatcgacgatagcgttcgccatgtgcagacgatcatcaacgttaaaaagcaggaatttatccagcgcgtgctgagcgatcagcattgtaatctgccgaaaagctttaagcagctgcactttagctgcctgaaagtgtttaacatgtttttcaacagcagcaacatctttgacaccgatacggacctgctgctggatatccatgaagcctttgtgagcccgccccaggtcccgaagtttaaaccccatattaagccgccccaccagctgcccgccaccctgcagccgccccaccagccccagcagatcatggtcaacaaaaagaaagtcgaaatggtttacaagagctaccatcacccctttaaggtttttacgctgcagaagaaacagagcagcggccacggcacgatgaatccccgtgcgagtatcctggccggtccgaatatcaaactgtgctttagttaa

SEQ ID NO: 127 - protein, 849 aa, Clarkia breweri
MRESLSSSSSNTQNLFLSTSPYDTAWLALIPHPHHHHHHGRPMFEKCLQWILHNQTPQGFWAAAGDNISDTDDDVTLDCLLSTLACLVALKRWQLAPDMIHKGLEFVNRNTERLVMKQKPSDVPRWFTIMFPAMLELAGASSLRVDFSENLNRILVELSQNRDDILTREEVDEKKQYSPLLLFLEALPAQSYDNDVLKQIIDKNLSNDGSLLQSPSATARAYMITGNTRCLSYLHSLTNSCSNGGVPSFYPVDDDLHDLVMVNQLTRSGLTEHLIPEIDHLLLKVQKNYKYKKASPKSLYSIAAELYRDSLAFWLLRVNNHWVSPSIFCWFLDDDEIRDHIETNYEEFAAVLLNVYRATDLMFSGEVQLVEARSFATKNLEKILATGNIHKTNADISSSLHKMIEHELRVPWTARMDHVENRIWIEEIASSALWFGKSSYLRLSCFHKMSLQQLAVKNYTLRQLVYRDELAEVERWSKERGLCDMGFCREKTGYCYYAFAASTCLPWSSDVRLVLTKAAVVITVADDFFDVEGSMVDLEKLTDAVRRWDAEGLGSHSKTIFEALDDLVNEVRLKCFQQNGQDIKNNLQQLWYETFHSWLMEAKWGKGLTSKPSVDVYLGNAMTSIAAHTMVLTASCLLGPGFPVHQLWSQRRHQDITSLLMVLTRLLNDIQSYLKEEDEGKINYVWMYMIENNQASIDDSVRHVQTIINVKKQEFIQRVLSDQHCNLPKSFKQLHFSCLKVFNMFFNSSNIFDTDTDLLLDIHEAFVSPPQVPKFKPHIKPPHQLPATLQPPHQPQQIMVNKKKVEMVYKSYHHPFKVFTLQKKQSSGHGTMNPRASILAGPNIKLCFS

SEQ ID NO: 128 - DNA, 43 bp, Artificial Sequence
  Primer
cacaaggagactgccatggcgaacacggcgaagcgtagtatcc

SEQ ID NO: 129 - DNA, 44 bp, Artificial Sequence
  Primer
gtctcctgtgtgaaattacatcaggcttttcagatactcatcgg

SEQ ID NO: 130 - DNA, 44 bp, Artificial Sequence
  Primer
cacaaggagactgccatgcgtcgtagtgcgaattaccagccgag

SEQ ID NO: 131 - DNA, 43 bp, Artificial Sequence
  Primer
gtctcctgtgtgaaattagtccagcgggatagggttaaacagc

SEQ ID NO: 132 - DNA, 48 bp, Artificial Sequence
  Primer
cacaaggagactgccatggagtttagcattagccagagtagttttgcg

SEQ ID NO: 133 - DNA, 45 bp, Artificial Sequence
  Primer
gtctcctgtgtgaaattaggcgtgcagcatactcttcatgtactc

SEQ ID NO: 134 - DNA, 42 bp, Artificial Sequence
  Primer
cacaaggagactgccatgtatagcctgcgtatttatgtggcg

SEQ ID NO: 135 - DNA, 46 bp, Artificial Sequence
  Primer
gtctcctgtgtgaaattaggcatagggttcaaacagcaggcaggcg

SEQ ID NO: 136 - DNA, 44 bp, Artificial Sequence
  Primer
cacaaggagactgccatgggttttagtcctgccttttatgcgtg

SEQ ID NO: 137 - DNA, 46 bp, Artificial Sequence
  Primer
gtctcctgtgtgaaattacaggggaaacgcttcaaacagcagactc

SEQ ID NO: 138 - DNA, 45 bp, Artificial Sequence
  Primer
cacaaggagactgccatggaactgaccctgacgagtctgagcccg

SEQ ID NO: 139 - DNA, 46 bp, Artificial Sequence
  Primer
gtctcctgtgtgaaattagcggcggttactcatcttcatgccatcc

SEQ ID NO: 140 - DNA, 43 bp, Artificial Sequence
  Primer
cacaaggagactgccatgtgtaccatcattagcgtcaatcatc

SEQ ID NO: 141 - DNA, 45 bp, Artificial Sequence
  Primer
gtctcctgtgtgaaattagacgtagggcttaaacagcagattggc

SEQ ID NO: 142 - DNA, 45 bp, Artificial Sequence
  Primer
cacaaggagactgccatggcgagtgcggtccccctgagtagtacg

SEQ ID NO: 143 - DNA, 47 bp, Artificial Sequence
  Primer
gtctcctgtgtgaaattaactactcagcaggggcgtaaaaaacaggg

SEQ ID NO: 144 - DNA, 45 bp, Artificial Sequence
  Primer
cacaaggagactgccatgcgtgagagcctgagcagtagcagtagc

SEQ ID NO: 145 - DNA, 44 bp, Artificial Sequence
  Primer
gtctcctgtgtgaaattaactaaagcacagtttgatattcggac

SEQ ID NO: 146 - DNA, 34 bp, Artificial Sequence
  Primer
ggcagtctccttgtgtgaaattgttatccgctca

SEQ ID NO: 147 - DNA, 35 bp, Artificial Sequence
  Primer
tttcacacaggagactgccatggattttccccagc

SEQ ID NO: 148 - DNA, 41 bp, Artificial Sequence
  Primer
atgtccaccgccgtgccctctatgcccactacccaaaaatg

SEQ ID NO: 149 - DNA, 42 bp, Artificial Sequence
  Primer
gcaggtcgactctagctatttgttgcgctggatgatgtaatc

SEQ ID NO: 150 - DNA, 40 bp, Artificial Sequence
  Primer
ggtacccggggatcctctagagatcgtttagatccgaagg

SEQ ID NO: 151 - DNA, 40 bp, Artificial Sequence
  Primer
cacggcggtggacattgtatgtcctcctggacttcgtggt

SEQ ID NO: 152 - DNA, 8564 bp, Artificial Sequence
  DNA encoding pVK9-P0480-optAaLINS-ispA*
gaggtctgcctcgtgaagaaggtgttgctgactcataccaggcctgaatcgccccatcatccagccagaaagtgagggagccacggttgatgagagctttgttgtaggtggacggggatcttttctacggggtctgacgctcagtggaacgaaaactcacgttaagggattttggtcatgagattatcaaaaaggatcatgcgagcaacctccataagatcagctaggcgatctttgggagcagtccttgtcgcgttacgaggtgagccggtggggaaccgttagctgcctatggtgtgagcccccctagagagcttcaagagcaatcagcccgacctagaaaggaggccaagagagagacctacggggggaaccgttttctgcctacgagatgggcacattactgggaagctttacggcgtcctcgtggaagttcaatgcccgcagacttaagtgctctattcacggtctgacgtgacacgctaaattcagacatagcttcattgattgtcggccacgagccagtctctccctcaacagtcataaaccaacctgcaatggtcaagcgatttcctttagctttcctagcttgtcgttgactggacttagctagtttttctcgctgtgctcgggcgtactcactgtttgggtctttccagcgttctgcggcctttttaccgccacgtcttcccatagtggccagagcttttcgccctcggctgctctgcgtctctgtctgacgagcagggacgactggctggcctttagcgacgtagccgcgcacacgtcgcgccatcgtctggcggtcacgcatcggcggcagatcaggctcacggccgtctgctccgaccgcctgagcgacggtgtaggcacgctcgtaggcgtcgatgatcttggtgtcttttaggcgctcaccagccgcttttaactggtatcccacagtcaaagcgtggcgaaaagccgtctcatcacgggcggcacgccctggagcagtccagaggacacggacgccgtcgatcagctctccagacgcttcagcggcgctcggcaggcttgcttcaagcgtggcaagtgcttttgcttccgcagtggcttttcttgccgcttcgatacgtgcccgtccgctagaaaactcctgctcatagcgttttttaggtttttctgtgcctgagatcatgcgagcaacctccataagatcagctaggcgatccacgcgattgtgctgggcatgccagcggtacgcggtgggatcgtcggagacgtgcagtggccaccggctcagcctatgtgaaaaagcctggtcagcgccgaaaacgcgggtcatttcctcggtcgttgcagccagcaggcgcatattcgggctgctcatgcctgctgcggcatacaccggatcaatgagccagatgagctggcatttcccgctcagtggattcacgccgatccaagctggcgctttttccaggcgtgcccagcgctccaaaatcgcgtagacctcggggtttacgtgctcgattttcccgccggcctggtggctcggcacatcaatgtccaggacaagcacggctgcgtgctgcgcgtgcgtcagagcaacatactggcaccgggcaagcgattttgaaccaactcggtataacttcggctgtgtttctcccgtgtccgggtctttgatccaagcgctggcgaagtcgcgggtcttgctgccctggaaattttctctgcccaggtgagcgaggaattcgcggcggtcttcgctcgtccagccacgtgatcgcagcgcgagctcgggatgggtgtcgaacagatcagcggaaaatttccaggccggtgtgtcaatgtctcgtgaatccgctagagtcatttttgagcgctttctcccaggtttggactgggggttagccgacgccctgtgagttaccgctcacggggcgttcaacatttttcaggtattcgtgcagcttatcgcttcttgccgcctgtgcgctttttcgacgcgcgacgctgctgccgattcggtgcaggtggtggcggcgctgacacgtcctgggcggccacggccacacgaaacgcggcatttacgatgtttgtcatgcctgcgggcaccgcgccacgatcgcggataattctcgctgccgcttccagctctgtgacgaccatggccaaaatttcgctcgggggacgcacttccagcgccatttgcgacctagccgcctccagctcctcggcgtggcgtttgttggcgcgctcgcggctggctgcggcacgacacgcatctgagcaatattttgcgcgccgtcctcgcgggtcaggccggggaggaatcaggccaccgcagtaggcgcaactgattcgatcctccactactgtgcgtcctcctggcgctgccgagcacgcagctcgtcagccagctcctcaagatccgccacgagagtttctaggtcgctcgcggcactggcccagtctcgtgatgctggcgcgtccgtcgtatcgagagctcggaaaaatccgatcaccgtttttaaatcgacggcagcatcgagcgcgtcggactccagcgcgacatcagagagatccatagctgatgattcgggccaattttggtacttcgtcgtgaaggtcatgacaccattataacgaacgttcgttaaagtttttggcggaaaatcacgcggcacgaaaattttcacgaagcgggactttgcgcagctcaggggtgctaaaaattttgtatcgcacttgatttttccgaaagacagattatctgcaaacggtgtgtcgtatttctggcttggtttttaaaaaatctggaatcgaaaatttgcggggcgaccgagaagttttttacaaaaggcaaaaactttttcgggatcagctaggcgatccacgcgattgtgctgggcatgccagcggtacgcggtgggatcgtcggagacgtgcagtggccaccggctcagcctatgtgaaaaagcctggtcagcgccgaaaacgcgggtcatttcctcggtcgttgcagccagcaggcgcatattcgggctgctcatgcctgctgcggcatacaccggatcggaccagttggtgattttgaacttttgctttgccacggaacggtctgcgttgtcgggaagatgcgtgatctgatccttcaactcagcaaaagttcgatttattcaacaaagccacgttgtgtctcaaaatctctgatgttacattgcacaagataaaaatatatcatcatgaacaataaaactgtctgcttacataaacagtaatacaaggggtgttatgagccatattcaacgggaaacgtcttgctcgaagccgcgattaaattccaacatggatgctgatttatatgggtataaatgggctcgcgataatgtcgggcaatcaggtgcgacaatctatcgattgtatgggaagcccgatgcgccagagttgtttctgaaacatggcaaaggtagcgttgccaatgatgttacagatgagatggtcagactaaactggctgacggaatttatgcctcttccgaccatcaagcattttatccgtactcctgatgatgcatggttactcaccactgcgatccccgggaaaacagcattccaggtattagaagaatatcctgattcaggtgaaaatattgttgatgcgctggcagtgttcctgcgccggttgcattcgattcctgtttgtaattgtccttttaacagcgatcgcgtatttcgtctcgctcaggcgcaatcacgaatgaataacggtttggttgatgcgagtgattttgatgacgagcgtaatggctggcctgttgaacaagtctggaaagaaatgcataagcttttgccattctcaccggattcagtcgtcactcatggtgatttctcacttgataaccttatttttgacgaggggaaattaataggttgtattgatgttggacgagtcggaatcgcagaccgataccaggatcttgccatcctatggaactgcctcggtgagttttctccttcattacagaaacggctttttcaaaaatatggtattgataatcctgatatgaataaattgcagtttcatttgatgctcgatgagtttttctaatcagaattggttaattggttgtaacactggcagagcattacgctgacttgacgggacggcggctttgttgaataaatcgcattcgccattcaggctgcgcaactgttgggaagggcgatcggtgcgggcctcttcgctattacgccagctggcgaaagggggatgtgctgcaaggcgattaagttgggtaacgccagggttttcccagtcacgacgttgtaaaacgacggccagtgaattcgagctcggtacccggggatcctctagagatcgtttagatccgaaggaaaacgtcgaaaagcaatttgcttttcgacgccccaccccgcgcgttttagcgtgtcagtagacgcgtagggtaagtggggtagcggcttgttagatatcttgaaatcggctttcaacagcattgatttcgatgtatttagctggccgttaccctgcgaatgtccacagggtagctggtagtttgaaaatcaacgccgttgcccttaggattcagtaactggcacattttgtaatgcgctagatctgtgtgcccagtcttccaggctgcttatcacagtgaaagcaaaaccaattcgtggctgcgaaagtcgtagccaccacgaagtccaggaggacatacaatgtccaccgccgtgccctctatgcccactacccaaaaatggtctattaccgaagacttagcctttattagcaatcccagcaaacaacataatcaccaaaccggctaccggatttttagtgacgaattttacctgaaacatgaaaacaaattgaaagatgtgcggcgcgccttgcgtgaagttgaagaaacccccctggaaggcttggtgatgattgacactttacagcggctgggtattgattaccactttcaaggcgaaattggtgccttgttacagaaacaacagcgcattagtacctgtgactatcccgaacatgatttgtttgaagtgagcactcgctttcgtctgttgcgtcaagaaggtcacaatgtgcccgccgacgtttttaataactttcgcgataaagaagggcgttttaaatctgaactgtcccgggatattcgcggattgatgtccttatacgaagccagtcaactgagcattcagggggaagacattttggatcaagccgctgacttttccagtcagttactgtctggatgggccaccaatttagatcatcaccaagcccgtctggtgcggaacgctttgacccatccctaccacaaaagtctggccacttttatggctcgcaactttaactacgattgcaaagggcaaaacggatgggtgaataacctgcaggaattggccaaaatggatttaaccatggttcaaagtatgcatcagaaagaagtgctgcaagttagccagtggtggaaagggcggggattggccaatgaactgaaattggtgcgcaaccaacccttgaaatggtatatgtggcccatggccgctttaaccgatccccggttttctgaagaacgcgtggaattgactaaacccatttcctttatttacattattgatgacatttttgacgtttatggcaccttagaagaattaaccctgtttactgatgccgtgaatcggtgggaattaactgctgttgaacagctgcccgactacatgaaaatttgttttaaagccttgtacgatattaccaacgaaattgcttacaaaatttacaaaaaacatgggcgcaaccccattgatagtttacgtcggacttgggccagcttatgcaatgcttttctggaagaagccaaatggtttgctagtggcaatttgcccaaagccgaagaatacctgaaaaacgggattattagctctggaatgcatgtggttaccgtgcacatgtttttcttgttaggcggttgttttactgaagaatccgtgaatttggttgatgaacatgccggcattacctccagtattgctactattttgcgtttatctgatgacttaggttccgccaaagatgaagaccaagatggctatgacggtagctacttggaatgttacctgaaagatcataaaggtagctctgtggaaaatgcccgtgaagaagttattcggatgatttccgatgcttggaaacgcttgaatgaagaatgcttatttcccaaccccttttctgccacctttcgcaaagggtccttaaatattgctcgtatggtgcccctgatgtacagttacgatgacaaccataacctgcccattctggaagaacacatgaaaaccatgttgtatgattccagtagctaatttcacacaggagactgccatggattttccccagcagctggaagcctgcgtgaaacaggccaaccaggccctgagccgctttatcgcccccctgccctttcagaacacccccgtggtggaaaccatgcagtacggcgccctgctgggcggcaaacgcctgcgcccctttctggtgtacgccaccggccacatgtttggcgtgagcaccaacaccctggatgcccccgccgccgccgtggaatgcatccacgcctactttctgatccacgatgatctgcccgccatggatgatgatgatctgcgccgcggcctgcccacctgccacgtgaaatttggcgaagccaacgccatcctggccggcgatgccctgcagaccctggcctttagcatcctgagcgatgccgatatgcccgaagtgagcgatcgcgatcgcatcagcatgatcagcgaactggccagcgccagcggcatcgccggcatgtgcggcggccaggccctggatctggatgccgaaggcaaacacgtgcccctggatgccctggaacgcatccaccgccacaaaaccggcgccctgatccgcgccgccgtgcgcctgggcgccctgagcgccggcgataaaggccgccgcgccctgcccgtgctggataaatacgccgaaagcatcggcctggcctttcaggtgcaggatgatatcctggatgtggtgggcgataccgccaccctgggcaaacgccagggcgccgatcagcagctgggcaaaagcacctaccccgccctgctgggcctggaacaggcccgcaaaaaagcccgcgatctgatcgatgatgcccgccagagcctgaaacagctggccgaacagagcctggataccagcgccctggaagccctggccgattacatcatccagcgcaacaaatagctagagtcgacctgcaggcatgcaagcttggcgtaatcatggtcatagctgtttcctgtgtgaaattgttatccgctcacaattccacacaacatacgagccggaagcataaagtgtaaagcctggggtgcctaatgagtgagctaactcacattaattgcgttgcgctcactgcccgctttccagtcgggaaacctgtcgtgccagctgcattaatgaatcggccaacgcgcggggagaggcggtttgcgtattggcgaacttttgctgagttgaaggatcagatcacgcatcttcccgacaacgcagaccgttccgtggcaaagcaaaagttcaaaatcagtaaccgtcagtgccgataagttcaaagttaaacctggtgttgataccaacattgaaacgctgatcgaaaacgcgctgaaaaacgctgctgaatgtgcgagcttcttccgcttcctcgctcactgactcgctgcgctcggtcgttcggctgcggcgagcggtatcagctcactcaaaggcggtaatacggttatccacagaatcaggggataacgcaggaaagaacatgtgagcaaaaggccagcaaaaggccaggaaccgtaaaaaggccgcgttgctggcgtttttccataggctccgcccccctgacgagcatcacaaaaatcgacgctcaagtcagaggtggcgaaacccgacaggactataaagataccaggcgtttccccctggaagctccctcgtgcgctctcctgttccgaccctgccgcttaccggatacctgtccgcctttctcccttcgggaagcgtggcgctttctcaatgctcacgctgtaggtatctcagttcggtgtaggtcgttcgctccaagctgggctgtgtgcacgaaccccccgttcagcccgaccgctgcgccttatccggtaactatcgtcttgagtccaacccggtaagacacgacttatcgccactggcagcagccactggtaacaggattagcagagcgaggtatgtaggcggtgctacagagttcttgaagtggtggcctaactacggctacactagaaggacagtatttggtatctgcgctctgctgaagccagttaccttcggaaaaagagttggtagctcttgatccggcaaacaaaccaccgctggtagcggtggtttttttgtttgcaagcagcagattacgcgcagaaaaaaaggatctcaagaagatcctttgatcttttctacggggtctgacgctcagtggaacgatccgtcga

SEQ ID NO: 153 - DNA, 55 bp, Artificial Sequence; identical to SEQ ID NO: 81
  Primer

SEQ ID NO: 154 - DNA, 54 bp, Artificial Sequence
  Primer
tccaatgtgaggttttagctactggaatcatacaacatggttttcatgtgttct

SEQ ID NO: 155 - DNA, 57 bp, Artificial Sequence
  Primer
aaggaattataaccaaatgtccaccgccgtgccctctatgcccactacccaaaaatg

SEQ ID NO: 156 - DNA, 55 bp, Artificial Sequence
  Primer
gatggggaagtttaggctagcctatttgttgcgctggatgatgtaatcggccagg

SEQ ID NO: 157 - DNA, 25 bp, Artificial Sequence
  Primer
ggaggattgggttaccctcagtgtg

SEQ ID NO: 158 - DNA, 25 bp, Artificial Sequence
  Primer
cgccatatcaatcccaacgctctgg

SEQ ID NO: 159 - DNA, 44 bp, Artificial Sequence
  Primer
ggaatattaagcttggtaccatgtccaccgccgtgccctctatg

SEQ ID NO: 160 - DNA, 42 bp, Artificial Sequence
  Primer
gtggatccgagctcggtaccctatttgttgcgctggatgatg

SEQ ID NO: 161 - protein, 609 aa, Solanum lycopersicum
MVSILSNIGMMVVTFKRPSLFTSLRRRSANNIIITKHSHPISTTRRSGNYKPTMWDFQFIQSLHNPYEGDKYMKRLNKLKKEVKKMMMTVEGSHDEELEKLELIDNLERLGVSYHFKDEIMQIMRSINININIAPPDSLYTTALKFRLLRQHGFHISQDILNDFKDENGNLKQSICKDTKDILNSSKDEHDNLKQSTCNNTKGLLKLYEASFLSIENESFLRNTTKSTLAHLMRYVDQNRCGEEDNMIVELVVHALELPRHWMVPRLETRWYISIYERMSNANPLLLELAKLDFNIVQATHQQDLRILSRWWKNTGLAEKLPFSRDILVENMFWAVGALFEPQHSYFRRLITKVIVFISIIDDIYDVYGTLDELELFTLAIQRWDTKAMEQLPDYMKVCYLALINIINEVAYEVLKNHDINVLPYLTKSWADLCKSYLQEAKWYHNGYKPNLEEYMDNARISIGVPMVLVHSLFLVTNQITKEALDSLTNYPDIIRWSATIFRLNDDLGTSSDELKRGDVSKSIQCYMNEKGASEEEAIEHIEFLIQETWEAMNTAQSKNSPLSETFIEVAKNITKASHFMYLHSDVKSSISKILFEPIIISNVAFALK

SEQ ID NO: 162 - protein, 594 aa, Backhousia citriodora; identical to SEQ ID NO: 72

SEQ ID NO: 163 - protein, 567 aa, Artemisia annua; identical to SEQ ID NO: 69

SEQ ID NO: 164 - protein, 583 aa, Artemisia annua
MASISLFPYSILKQTSPLARGTAYNRIYSTKTTGITVDVAESHVRRSANYEPSSWSFDHIQSLSSKYTGDDCVARANTLKESVKTMIRKEGNLLRTLELVDELQRLGISYLFEGEISNLLETIYYNHYKFPEKWNKFDLNLKALGFRLLRQHGYHVPQEIFLNFKDKNQNLNSYLLEDVVGMLNLYEASYHSFEDESILTEARDIATKYLKASLEKIDGSILSLVSHALDNRLHWRVPRVESKWFIEVYEKRVGASPTLIELAKLDFDMVQAIHLEDLKHASRWWRNTSWDTKLTFARDMLVENFLWTVGFSYLPNFSHGRRTITKVAAMITTLDDVYDVFGTLGELEQFTDVINRWDIKAIEQLPDYMKICFFGLYNSINDITYETLATKGFLILPYIKKAWADLCKSYLVEAQWYHRGHIPTLNEYLDNACVSISGPVALMHVHFLTSVSSTKEIHHCIERTQNIVRYVSLIFRLTDDLGTSLGEMERGDTLKSIQLYMHETGATEPEARSYIKSLIDKTWKKLNKERAIVSSESSREFIDYATNLARMAHFMYGEGDEDFRLDVIKSHVSSLLFTPIQGI

SEQ ID NO: 165 - protein, 574 aa, Actinidia arguta; identical to SEQ ID NO: 1

SEQ ID NO: 166 - protein, 574 aa, Actinidia polygama
MASFHRFCVSSLLVPNNSPQISNAYRAPAVPSMPTTQKWSITEDLAFISNPSKQHNHQTGYRTFSDEFYVKREKKLKDVRRALREVEETPLEGLVMIDTLQRLGIDYHFQGEIGALLQKQQRKSKCDYPEHDLFEVSTRFRLLRQEGHNVPADVFNHFRDKKGRFKSELSRDIRGLMSLYEASQLSIQGEDILDQAADFSSQLLSGWATNPDHHQARLVRNALTHPYHKSLATFTARNFHYDCKGQNGWVNNLQELAKMDLTVVQSMHQKEVLQVSQWWKDRGLANELKLVRNQPLKWYMWPMAALTDPRFSEERVELTKPISFIYIIDDIFDVYGTLEELTLFTDAVNRWELTAVEQLPDYMKVCFKALYDITNEIAYKIYKKHGWNPIDSLRRMWASLCNAFLVEAKWFASGHLPKAEEYLKNGIISSGMHVVTVHMFFLLGGCFTDESVNLVDEHAGITSSIATILRLSDDLGSAKDEDQDGYDGSYVEYYLKDHKGSSVENAREEVIRMISDAWKRLNEECLSPNPFSATFRKGCLNIARMVPLMYSYDDNHNLPLLEEHMKAMLYDSSS

SEQ ID NO: 167 - protein, 604 aa, Perilla frutescens var. hirtella
MSSMRIYVAIMKKPSVKHVDYVDKKASKPSWRVSSSATAGLRASSSLQLDVKKPADEILTARRSGNYQPSLWDFNYLQSLNTTHYKEERHLKREAELIEQVKMLLDEEMGAVQKLDLVDDLKNLGLSYFFEDQIKQILTFIYNEHECFRSNVEAKERDLYFTALGFRLLRQHGFQVSQEVFDCFKNEEGSDFKASLGDDTKGLVQLYEASFLLREGEDTLELARQYATKFLQKKVDHELIDDDSNLLSWIRHSLEIPLHWRIQRLEARWFLDAYATRHDVNPIILELAKLDFNIIQATQQEELKDLSRWWNSTCLVEKLPFVRDRLVESYFWAIALFEPHQYGYHRKIAAKIITLITSLDDVYDIYGTLDELQLFTDAIQRWDTESISRLAYYMQLFYMVLYNFVSELAYDGLKEKGFITIPYLQRSWADLVEAYLKEAKWFYNGYTPSMEEYLNNAYISIGATPVISQVFFTLATSIDKPVIESLYEYHRILRLSGMLVRLPDDLGTSPFEMKRGDVPKTIELYMKERNATEIEAQEHVRFLIREAWREMNTATAAADCPFTDDLVAAAANLGRAAQFMYLDGDGNHSQLHQRIASLLFEPYA

SEQ ID NO: 168 - protein, 603 aa, Perilla setoensis
MSSMRTYVAIMKKPSVEHVDNVDKKASKPSWRVSLSAGLRSSCSLQLEVKPADQILTARRSGNYQPSLWDFNYLQSLNTTHYKEVRHLKREAELIEQVKMLLEEEMEAVQQLELVDDLKNLGLSYFFEDQIKQILTFIYNEHKCFHSNSIIEAEEIRDLYFTALGFRLLRQHGFQISQEVFDCFKNEEGSDFKARLGDDTKGLLQLYEASFLLREGEDTLELARQYATKFLQKKVDHELIDDNNLLSWILHSLEIPLHWRIQRLEARWFLDAYASRRDMNQIILELAKLDFNIIQATQQEELKDLSRWWKSSCLAEKLPFVRDRLVESYFWAIALFEPHQYGYHRKIAAKIITLITSLDDVYDIYGTLDELQLFTDAIQRWDTESISRLPYYMQLFYMVLYNFVPRLAYDGLKEKGFITIPYLQRSWADLVEAYLKEAKWYYNGYTPSMEEYLNNAYISIGATPVISQVFFTLATSIDKPVIDSLYEYHRILRLSGILVRLPDDLGTSPFEMKRGDVPKAIQLYMKERNATEIEAQEHVRFLIREAWKEMNTATAAVDCPFTDDLVTAAANLGRAAQFMYLDGDGNHSQLHQRIACLLFEPYA

SEQ ID NO: 169 - protein, 547 aa, Arabidopsis thaliana; identical to SEQ ID NO: 105

SEQ ID NO: 170 - DNA, 1644 bp, Arabidopsis thaliana; identical to SEQ ID NO: 90

SEQ ID NO: 171 - DNA, 1644 bp, Artificial Sequence; identical to SEQ ID NO: 104
  DNA having modified codons, which encodes linalool synthase gene derived from Arabidopsis thaliana

SEQ ID NO: 172 - protein, 607 aa, Perilla frutescens var. crispa; identical to SEQ ID NO: 115

SEQ ID NO: 173 - DNA, 1824 bp, Perilla frutescens var. crispa; identical to SEQ ID NO: 95

SEQ ID NO: 174 - DNA, 1824 bp, Artificial Sequence; identical to SEQ ID NO: 114
  DNA having modified codons, which encodes linalool synthase gene derived from Pereilla frutescens var. crispa

SEQ ID NO: 175 - protein, 602 aa, Vitis vinifera; identical to SEQ ID NO: 119

SEQ ID NO: 176 - DNA, 1809 bp, Vitis vinifera; identical to SEQ ID NO: 97

SEQ ID NO: 177 - DNA, 1809 bp, Artificial Sequence; identical to SEQ ID NO: 118
  DNA having modified codons, which encodes linalool synthase gene derived from Vitis vinifera

SEQ ID NO: 178 - protein, 606 aa, Mentha citrata; identical to SEQ ID NO: 123

SEQ ID NO: 179 - DNA, 1821 bp, Mentha citrata; identical to SEQ ID NO: 99

SEQ ID NO: 180 - DNA, 1821 bp, Artificial Sequence; identical to SEQ ID NO: 122
  DNA having modified codons, which encodes linalool synthase gene derived from Mentha citrata

SEQ ID NO: 181 - protein, 535 aa, Ocimum basilicum; identical to SEQ ID NO: 125

SEQ ID NO: 182 - DNA, 1608 bp, Ocimum basilicum; identical to SEQ ID NO: 100

SEQ ID NO: 183 - DNA, 1608 bp, Artificial Sequence; identical to SEQ ID NO: 124
  DNA having modified codons, which encodes linalool synthase gene derived from Ocimum basilicum